European Patent Specification EP 4 001 298 B1, published March 5, 2025. Title: POLYVALENT IMMUNOGENICITY COMPOSITION FOR HUMAN PAPILLOMAVIRUS. Applicant: SinoCellTech Ltd. The sequence listing filed with the application follows.

SEQUENCE LISTING (162 sequences)

SEQ ID NO: 1 - protein, 469 aa, Homo sapiens
  0601 Amino acid sequence of HPV type 6 L1 protein aa 1-469
MWRPSDSTVYVPPPNPVSKVVATDAYVTRTNIFYHASSSRLLAVGHPYFSIKRANKTVVPKVSGYQYRVFKVVLPDPNKFALPDSSLFDPTTQRLVWACTGLEVGRGQPLGVGVSGHPFLNKYDDVENSGSGGNPGQDNRVNVGMDYKQTQLCMVGCAPPLGEHWGKGKQCTNTPVQAGDCPPLELITSVIQDGDMVDTGFGAMNFADLQTNKSDVPIDICGTTCKYPDYLQMAADPYGDRLFFFLRKEQMFARHFFNRAGEVGEPVPDTLIIKGSGNRTSVGSSIYVNTPSGSLVSSEAQLFNKPYWLQKAQGHNNGICWGNQLFVTVVDTTRSTNMTLCASVTTSSTYTNSDYKEYMRHVEEYDLQFIFQLCSITLSAEVMAYIHTMNPSVLEDWNFGLSPPPNGTLEDTYRYVQSQAITCQKPTPEKEKPDPYKNLSFWEVNLKEKFSSELDQYPLGRKFLLQSGY

SEQ ID NO: 2 - protein, 26 aa, Homo sapiens
  0602 Amino acid sequence of HPV type 33 L1 protein aa 474-499
KAKPKLKRAAPTSTRTSSAKRKKVKK

SEQ ID NO: 3 - protein, 495 aa, Artificial sequence
  0603 Amino acid sequence of chimeric HPV type 6 L1 protein
MWRPSDSTVYVPPPNPVSKVVATDAYVTRTNIFYHASSSRLLAVGHPYFSIKRANKTVVPKVSGYQYRVFKVVLPDPNKFALPDSSLFDPTTQRLVWACTGLEVGRGQPLGVGVSGHPFLNKYDDVENSGSGGNPGQDNRVNVGMDYKQTQLCMVGCAPPLGEHWGKGKQCTNTPVQAGDCPPLELITSVIQDGDMVDTGFGAMNFADLQTNKSDVPIDICGTTCKYPDYLQMAADPYGDRLFFFLRKEQMFARHFFNRAGEVGEPVPDTLIIKGSGNRTSVGSSIYVNTPSGSLVSSEAQLFNKPYWLQKAQGHNNGICWGNQLFVTVVDTTRSTNMTLCASVTTSSTYTNSDYKEYMRHVEEYDLQFIFQLCSITLSAEVMAYIHTMNPSVLEDWNFGLSPPPNGTLEDTYRYVQSQAITCQKPTPEKEKPDPYKNLSFWEVNLKEKFSSELDQYPLGRKFLLQSGYKAKPKLKRAAPTSTRTSSAKRKKVKK

SEQ ID NO: 4 - DNA, 1488 bp, Artificial sequence
  0604 Nucleotide sequence of chimeric HPV type 6 L1 protein
atgtggagaccatctgacagcacagtctatgtgcctcctccaaaccctgtgagcaaggtggtggctacagatgcctatgtgaccaggaccaacatcttctaccatgcctcctccagcagactgctggctgtgggacacccatacttcagcatcaagagggctaacaagacagtggtgccaaaggtgtctggctaccaatacagggtgttcaaggtggtgctgcctgacccaaacaagtttgccctgcctgactcctccctgtttgacccaaccacccagagactggtgtgggcttgtactggattggaggtgggcaggggacaaccactgggagtgggagtgtctggacacccattcctgaacaaatatgatgatgtggagaactctggctctggaggcaaccctggacaagacaacagggtgaatgtggggatggactacaagcagacccaactttgtatggtgggctgtgcccctccactgggagaacactggggcaagggcaagcagtgtaccaacacacctgtccaggctggagactgtcctccattggaactgattacctctgtgattcaggatggagatatggtggacacaggctttggagctatgaactttgctgacctccaaaccaacaagtctgatgtgccaattgacatctgtggcaccacttgtaaataccctgactacctccaaatggctgctgacccatatggagacagactgttcttcttcctgaggaaggaacagatgtttgccagacacttcttcaacagggctggagaggtgggagaacctgtgcctgacaccctgattatcaagggctctggcaacaggacctctgtgggctccagcatctatgtgaacacaccatctggctccctggtgtcctctgaggctcaacttttcaacaagccatactggctccaaaaggctcaaggacacaacaatggcatctgttggggcaaccaactttttgtgacagtggtggacaccaccaggagcaccaatatgaccctgtgtgcctctgtgaccacctccagcacctacaccaactctgactacaaggaatatatgaggcatgtggaggaatatgacctccaattcatcttccaactttgtagcatcaccctgtctgctgaggtgatggcttacatccacacaatgaacccatctgtgttggaggactggaactttggactgagccctcctccaaatggcaccttggaggacacctacagatatgtccagagccaggctatcacttgtcagaagccaacacctgagaaggagaagcctgacccatacaagaacctgtccttctgggaggtgaacctgaaagagaagttctcctctgaactggaccaatacccactgggcaggaagttcctgctccaatctggctacaaagccaagccaaaactgaaaagggctgccccaaccagcaccaggacctcctctgccaagaggaagaaggtgaagaagtaa

SEQ ID NO: 5 - DNA, 1522 bp, Artificial sequence
  0605 Synthetic HPV6 L1 gene
ctgggtaccatgtggagaccatctgacagcacagtctatgtgcctcctccaaaccctgtgagcaaggtggtggctacagatgcctatgtgaccaggaccaacatcttctaccatgcctcctccagcagactgctggctgtgggacacccatacttcagcatcaagagggctaacaagacagtggtgccaaaggtgtctggctaccaatacagggtgttcaaggtggtgctgcctgacccaaacaagtttgccctgcctgactcctccctgtttgacccaaccacccagagactggtgtgggcttgtactggattggaggtgggcaggggacaaccactgggagtgggagtgtctggacacccattcctgaacaaatatgatgatgtggagaactctggctctggaggcaaccctggacaagacaacagggtgaatgtggggatggactacaagcagacccaactttgtatggtgggctgtgcccctccactgggagaacactggggcaagggcaagcagtgtaccaacacacctgtccaggctggagactgtcctccattggaactgattacctctgtgattcaggatggagatatggtggacacaggctttggagctatgaactttgctgacctccaaaccaacaagtctgatgtgccaattgacatctgtggcaccacttgtaaataccctgactacctccaaatggctgctgacccatatggagacagactgttcttcttcctgaggaaggaacagatgtttgccagacacttcttcaacagggctggagaggtgggagaacctgtgcctgacaccctgattatcaagggctctggcaacaggacctctgtgggctccagcatctatgtgaacacaccatctggctccctggtgtcctctgaggctcaacttttcaacaagccatactggctccaaaaggctcaaggacacaacaatggcatctgttggggcaaccaactttttgtgacagtggtggacaccaccaggagcaccaatatgaccctgtgtgcctctgtgaccacctccagcacctacaccaactctgactacaaggaatatatgaggcatgtggaggaatatgacctccaattcatcttccaactttgtagcatcaccctgtctgctgaggtgatggcttacatccacacaatgaacccatctgtgttggaggactggaactttggactgagccctcctccaaatggcaccttggaggacacctacagatatgtccagagccaggctatcacttgtcagaagccaacacctgagaaggagaagcctgacccatacaagaacctgtccttctgggaggtgaacctgaaagagaagttctcctctgaactggaccaatacccactgggcaggaagttcctgctccaatctggctacaggggcaggtccagcatcaggacaggagtgaagagacctgctgtgagcaaggcatctgctgccccaaagaggaagagggctaagaccaagaggtaaactcgagctc

SEQ ID NO: 6 - DNA, 1519 bp, Artificial sequence
  0606 Synthetic HPV33 L1 gene
ctgggtaccatgagtgtgtggagaccatctgaggctacagtctacctgcctcctgtgcctgtgagcaaggtggtgagcacagatgaatatgtgagcaggaccagcatctactactatgctggctccagcagactgctggctgtgggacacccatacttcagcatcaagaacccaaccaatgccaagaaactgctggtgccaaaggtgtctggactccaatacagggtgttcagggtgagactgcctgacccaaacaagtttggctttcctgacacctccttctacaaccctgacacccagagactggtgtgggcttgtgtgggattggagattggcaggggacaaccactgggagtgggcatctctggacacccactgctgaacaagtttgatgacacagagacaggcaacaaataccctggacaacctggagcagacaacagggagtgtctgagtatggactacaagcagacccaactttgtctgctgggctgtaagcctccaacaggagaacactggggcaagggagtggcttgtaccaatgctgcccctgccaatgactgtcctccattggaactgataaacaccatcattgaggatggagatatggtggacacaggctttggctgtatggacttcaagaccctccaagccaacaagtctgatgtgccaattgacatctgtggcagcacttgtaaataccctgactacctgaaaatgacctctgaaccatatggagactccctgttcttcttcctgaggagggaacagatgtttgtgagacacttcttcaacagggctggcaccctgggagaggctgtgcctgatgacctctacatcaagggctctggcaccacagccagcatccagtcctctgccttctttccaacaccatctggcagtatggtgacctctgagagccaacttttcaacaagccatactggctccaaagggctcaaggacacaacaatggcatctgttggggcaaccaggtgtttgtgacagtggtggacaccaccaggagcaccaatatgaccctgtgtacccaggtgacctctgacagcacctacaagaatgagaacttcaaggaatacatcaggcatgtggaggaatatgacctccaatttgtgttccaactttgtaaggtgaccctgacagcagaggtgatgacctacatccatgctatgaaccctgacatcttggaggactggcagtttggactgacacctcctccatctgcctccctccaagacacctacaggtttgtgaccagccaggctatcacttgtcagaagacagtgcctccaaaggagaaggaggacccactgggcaaatacaccttctgggaggtggacctgaaagagaagttctctgctgacctggaccagtttccactgggcaggaagttcctgctccaagcaggactgaaagccaagccaaaactgaaaagggctgccccaaccagcaccaggacctcctctgccaagaggaagaaggtgaagaagtaaactcgagctc

SEQ ID NO: 7 - DNA, 35 bp, Artificial sequence
  0607 HPV6L1 F1
cttggtaccatgtggagaccatctgacagcacagt

SEQ ID NO: 8 - DNA, 36 bp, Artificial sequence
  0608 HPV6L1 R1
gcttggctttgtagccagattggagcaggaacttcc

SEQ ID NO: 9 - DNA, 1426 bp, Artificial sequence
  0609 HPV6L1 amplified sequence 1
cttggtaccatgtggagaccatctgacagcacagtctatgtgcctcctccaaaccctgtgagcaaggtggtggctacagatgcctatgtgaccaggaccaacatcttctaccatgcctcctccagcagactgctggctgtgggacacccatacttcagcatcaagagggctaacaagacagtggtgccaaaggtgtctggctaccaatacagggtgttcaaggtggtgctgcctgacccaaacaagtttgccctgcctgactcctccctgtttgacccaaccacccagagactggtgtgggcttgtactggattggaggtgggcaggggacaaccactgggagtgggagtgtctggacacccattcctgaacaaatatgatgatgtggagaactctggctctggaggcaaccctggacaagacaacagggtgaatgtggggatggactacaagcagacccaactttgtatggtgggctgtgcccctccactgggagaacactggggcaagggcaagcagtgtaccaacacacctgtccaggctggagactgtcctccattggaactgattacctctgtgattcaggatggagatatggtggacacaggctttggagctatgaactttgctgacctccaaaccaacaagtctgatgtgccaattgacatctgtggcaccacttgtaaataccctgactacctccaaatggctgctgacccatatggagacagactgttcttcttcctgaggaaggaacagatgtttgccagacacttcttcaacagggctggagaggtgggagaacctgtgcctgacaccctgattatcaagggctctggcaacaggacctctgtgggctccagcatctatgtgaacacaccatctggctccctggtgtcctctgaggctcaacttttcaacaagccatactggctccaaaaggctcaaggacacaacaatggcatctgttggggcaaccaactttttgtgacagtggtggacaccaccaggagcaccaatatgaccctgtgtgcctctgtgaccacctccagcacctacaccaactctgactacaaggaatatatgaggcatgtggaggaatatgacctccaattcatcttccaactttgtagcatcaccctgtctgctgaggtgatggcttacatccacacaatgaacccatctgtgttggaggactggaactttggactgagccctcctccaaatggcaccttggaggacacctacagatatgtccagagccaggctatcacttgtcagaagccaacacctgagaaggagaagcctgacccatacaagaacctgtccttctgggaggtgaacctgaaagagaagttctcctctgaactggaccaatacccactgggcaggaagttcctgctccaatctggctacaaagccaagc

SEQ ID NO: 10 - DNA, 35 bp, Artificial sequence
  0610 HPV6L1 F2
atctggctacaaagccaagccaaaactgaaaaggg

SEQ ID NO: 11 - DNA, 37 bp, Artificial sequence
  0611 HPV6L1 R2
ctgtctagatttacttcttcaccttcttcctcttggc

SEQ ID NO: 12 - DNA, 101 bp, Artificial sequence
  0612 HPV6L1 amplified sequence 2
atctggctacaaagccaagccaaaactgaaaagggctgccccaaccagcaccaggacctcctctgccaagaggaagaaggtgaagaagtaaatctagacag

SEQ ID NO: 13 - protein, 38 aa, Homo sapiens
  0613 Amino acid sequence of HPV type 59 L1 protein aa 471-508
LQLGARPKPTIGPRKRAAPAPTSTPSPKRVKRRKSSRK

SEQ ID NO: 14 - protein, 470 aa, Homo sapiens
  1101 Amino acid sequence of HPV type 11 L1 protein aa 1-470
MWRPSDSTVYVPPPNPVSKVVATDAYVKRTNIFYHASSSRLLAVGHPYYSIKKVNKTVVPKVSGYQYRVFKVVLPDPNKFALPDSSLFDPTTQRLVWACTGLEVGRGQPLGVGVSGHPLLNKYDDVENSGGYGGNPGQDNRVNVGMDYKQTQLCMVGCAPPLGEHWGKGTQCSNTSVQNGDCPPLELITSVIQDGDMVDTGFGAMNFADLQTNKSDVPLDICGTVCKYPDYLQMAADPYGDRLFFYLRKEQMFARHFFNRAGTVGEPVPDDLLVKGGNNRSSVASSIYVHTPSGSLVSSEAQLFNKPYWLQKAQGHNNGICWGNHLFVTVVDTTRSTNMTLCASVSKSATYTNSDYKEYMRHVEEFDLQFIFQLCSITLSAEVMAYIHTMNPSVLEDWNFGLSPPPNGTLEDTYRYVQSQAITCQKPTPEKEKQDPYKDMSFWEVNLKEKFSSELDQFPLGRKFLLQSGY

SEQ ID NO: 15 - protein, 26 aa, Homo sapiens
  1102 Amino acid sequence of HPV type 33 L1 protein aa 474-499
KAKPKLKRAAPTSTRTSSAKRKKVKK

SEQ ID NO: 16 - protein, 496 aa, Artificial sequence
  1103 Amino acid sequence of chimeric HPV type 11 L1 protein
MWRPSDSTVYVPPPNPVSKVVATDAYVKRTNIFYHASSSRLLAVGHPYYSIKKVNKTVVPKVSGYQYRVFKVVLPDPNKFALPDSSLFDPTTQRLVWACTGLEVGRGQPLGVGVSGHPLLNKYDDVENSGGYGGNPGQDNRVNVGMDYKQTQLCMVGCAPPLGEHWGKGTQCSNTSVQNGDCPPLELITSVIQDGDMVDTGFGAMNFADLQTNKSDVPLDICGTVCKYPDYLQMAADPYGDRLFFYLRKEQMFARHFFNRAGTVGEPVPDDLLVKGGNNRSSVASSIYVHTPSGSLVSSEAQLFNKPYWLQKAQGHNNGICWGNHLFVTVVDTTRSTNMTLCASVSKSATYTNSDYKEYMRHVEEFDLQFIFQLCSITLSAEVMAYIHTMNPSVLEDWNFGLSPPPNGTLEDTYRYVQSQAITCQKPTPEKEKQDPYKDMSFWEVNLKEKFSSELDQFPLGRKFLLQSGYKAKPKLKRAAPTSTRTSSAKRKKVKK

SEQ ID NO: 17 - DNA, 1492 bp, Artificial sequence
  1104 Nucleotide sequence of chimeric HPV type 11 L1 protein
atgtggagaccatctgacagcacagtctatgtgcctcctccaaaccctgtgagcaaggtggtggctacagatgcctatgtgaagaggaccaacatcttctaccatgcctcctccagcagactgctggctgtgggacacccatactacagcatcaagaaggtgaacaagacagtggtgccaaaggtgtctggctaccaatacagggtgttcaaggtggtgctgcctgacccaaacaagtttgccctgcctgactcctccctgtttgacccaaccacccagagactggtgtgggcttgtactggattggaggtgggcaggggacaaccactgggagtgggagtgtctggacacccactgctgaacaaatatgatgatgtggagaactctggaggctatggaggcaaccctggacaagacaacagggtgaatgtggggatggactacaagcagacccaactttgtatggtgggctgtgcccctccactgggagaacactggggcaagggcacccagtgtagcaacacctctgtccagaatggagactgtcctccattggaactgattacctctgtgattcaggatggagatatggtggacacaggctttggagctatgaactttgctgacctccaaaccaacaagtctgatgtgccactggacatctgtggcacagtgtgtaaataccctgactacctccaaatggctgctgacccatatggagacagactgttcttctacctgaggaaggaacagatgtttgccagacacttcttcaacagggctggcacagtgggagaacctgtgcctgatgacctgctggtgaagggaggcaacaacaggtcctctgtggcatccagcatctatgtgcatacaccatctggctccctggtgtcctctgaggctcaacttttcaacaagccatactggctccaaaaggctcaaggacacaacaatggcatctgttggggcaaccacctgtttgtgacagtggtggacaccaccaggagcaccaatatgaccctgtgtgcctctgtgagcaagtctgccacctacaccaactctgactacaaggaatatatgaggcatgtggaggagtttgacctccaattcatcttccaactttgtagcatcaccctgtctgctgaggtgatggcttacatccacacaatgaacccatctgtgttggaggactggaactttggactgagccctcctccaaatggcaccttggaggacacctacagatatgtccagagccaggctatcacttgtcagaagccaacacctgagaaggagaagcaggacccatacaaggatatgagtttctgggaggtgaacctgaaagagaagttctcctctgaactggaccagtttccactgggcaggaagttcctgctccaatctggctacaaagccaagccaaaactgaaaagggctgccccaaccagcaccaggacctcctctgccaagaggaagaaggtgaagaagtaaa

SEQ ID NO: 18 - DNA, 1525 bp, Artificial sequence
  1105 Synthetic HPV11 L1 gene
ctgggtaccatgtggagaccatctgacagcacagtctatgtgcctcctccaaaccctgtgagcaaggtggtggctacagatgcctatgtgaagaggaccaacatcttctaccatgcctcctccagcagactgctggctgtgggacacccatactacagcatcaagaaggtgaacaagacagtggtgccaaaggtgtctggctaccaatacagggtgttcaaggtggtgctgcctgacccaaacaagtttgccctgcctgactcctccctgtttgacccaaccacccagagactggtgtgggcttgtactggattggaggtgggcaggggacaaccactgggagtgggagtgtctggacacccactgctgaacaaatatgatgatgtggagaactctggaggctatggaggcaaccctggacaagacaacagggtgaatgtggggatggactacaagcagacccaactttgtatggtgggctgtgcccctccactgggagaacactggggcaagggcacccagtgtagcaacacctctgtccagaatggagactgtcctccattggaactgattacctctgtgattcaggatggagatatggtggacacaggctttggagctatgaactttgctgacctccaaaccaacaagtctgatgtgccactggacatctgtggcacagtgtgtaaataccctgactacctccaaatggctgctgacccatatggagacagactgttcttctacctgaggaaggaacagatgtttgccagacacttcttcaacagggctggcacagtgggagaacctgtgcctgatgacctgctggtgaagggaggcaacaacaggtcctctgtggcatccagcatctatgtgcatacaccatctggctccctggtgtcctctgaggctcaacttttcaacaagccatactggctccaaaaggctcaaggacacaacaatggcatctgttggggcaaccacctgtttgtgacagtggtggacaccaccaggagcaccaatatgaccctgtgtgcctctgtgagcaagtctgccacctacaccaactctgactacaaggaatatatgaggcatgtggaggagtttgacctccaattcatcttccaactttgtagcatcaccctgtctgctgaggtgatggcttacatccacacaatgaacccatctgtgttggaggactggaactttggactgagccctcctccaaatggcaccttggaggacacctacagatatgtccagagccaggctatcacttgtcagaagccaacacctgagaaggagaagcaggacccatacaaggatatgagtttctgggaggtgaacctgaaagagaagttctcctctgaactggaccagtttccactgggcaggaagttcctgctccaatctggctacaggggcaggacctctgccaggacaggcatcaagagacctgctgtgagcaagccaagcacagccccaaagaggaagaggaccaagaccaagaagtaaactcgagctc

SEQ ID NO: 19 - DNA, 1519 bp, Artificial sequence; identical to SEQ ID NO: 6
  1106 Synthetic HPV33 L1 gene

SEQ ID NO: 20 - DNA, 35 bp, Artificial sequence; identical to SEQ ID NO: 7
  1107 HPV11L1 F1

SEQ ID NO: 21 - DNA, 36 bp, Artificial sequence; identical to SEQ ID NO: 8
  1108 HPV11L1 R1

SEQ ID NO: 22 - DNA, 1429 bp, Artificial sequence
  1109 HPV11L1 amplified sequence 1
cttggtaccatgtggagaccatctgacagcacagtctatgtgcctcctccaaaccctgtgagcaaggtggtggctacagatgcctatgtgaagaggaccaacatcttctaccatgcctcctccagcagactgctggctgtgggacacccatactacagcatcaagaaggtgaacaagacagtggtgccaaaggtgtctggctaccaatacagggtgttcaaggtggtgctgcctgacccaaacaagtttgccctgcctgactcctccctgtttgacccaaccacccagagactggtgtgggcttgtactggattggaggtgggcaggggacaaccactgggagtgggagtgtctggacacccactgctgaacaaatatgatgatgtggagaactctggaggctatggaggcaaccctggacaagacaacagggtgaatgtggggatggactacaagcagacccaactttgtatggtgggctgtgcccctccactgggagaacactggggcaagggcacccagtgtagcaacacctctgtccagaatggagactgtcctccattggaactgattacctctgtgattcaggatggagatatggtggacacaggctttggagctatgaactttgctgacctccaaaccaacaagtctgatgtgccactggacatctgtggcacagtgtgtaaataccctgactacctccaaatggctgctgacccatatggagacagactgttcttctacctgaggaaggaacagatgtttgccagacacttcttcaacagggctggcacagtgggagaacctgtgcctgatgacctgctggtgaagggaggcaacaacaggtcctctgtggcatccagcatctatgtgcatacaccatctggctccctggtgtcctctgaggctcaacttttcaacaagccatactggctccaaaaggctcaaggacacaacaatggcatctgttggggcaaccacctgtttgtgacagtggtggacaccaccaggagcaccaatatgaccctgtgtgcctctgtgagcaagtctgccacctacaccaactctgactacaaggaatatatgaggcatgtggaggagtttgacctccaattcatcttccaactttgtagcatcaccctgtctgctgaggtgatggcttacatccacacaatgaacccatctgtgttggaggactggaactttggactgagccctcctccaaatggcaccttggaggacacctacagatatgtccagagccaggctatcacttgtcagaagccaacacctgagaaggagaagcaggacccatacaaggatatgagtttctgggaggtgaacctgaaagagaagttctcctctgaactggaccagtttccactgggcaggaagttcctgctccaatctggctacaaagccaagc

SEQ ID NO: 23 - DNA, 35 bp, Artificial sequence; identical to SEQ ID NO: 10
  1110 HPV11L1 F2

SEQ ID NO: 24 - DNA, 37 bp, Artificial sequence; identical to SEQ ID NO: 11
  1111 HPV11L1 R2

SEQ ID NO: 25 - DNA, 101 bp, Artificial sequence; identical to SEQ ID NO: 12
  1112 HPV11L1 amplified sequence 2

SEQ ID NO: 26 - protein, 38 aa, Homo sapiens; identical to SEQ ID NO: 13
  1113 Amino acid sequence of HPV type 59 L1 protein aa 471-508

SEQ ID NO: 27 - protein, 474 aa, Homo sapiens
  1601 Amino acid sequence of HPV type 16 L1 protein aa 1-474
MSLWLPSEATVYLPPVPVSKVVSTDEYVARTNIYYHAGTSRLLAVGHPYFPIKKPNNNKILVPKVSGLQYRVFRIHLPDPNKFGFPDTSFYNPDTQRLVWACVGVEVGRGQPLGVGISGHPLLNKLDDTENASAYAANAGVDNRECISMDYKQTQLCLIGCKPPIGEHWGKGSPCTNVAVNPGDCPPLELINTVIQDGDMVDTGFGAMDFTTLQANKSEVPLDICTSICKYPDYIKMVSEPYGDSLFFYLRREQMFVRHLFNRAGAVGENVPDDLYIKGSGSTANLASSNYFPTPSGSMVTSDAQIFNKPYWLQRAQGHNNGICWGNQLFVTVVDTTRSTNMSLCAAISTSETTYKNTNFKEYLRHGEEYDLQFIFQLCKITLTADVMTYIHSMNSTILEDWNFGLQPPPGGTLEDTYRFVTSQAIACQKHTPPAPKEDPLKKYTFWEVNLKEKFSADLDQFPLGRKFLLQAGL

SEQ ID NO: 28 - protein, 26 aa, Homo sapiens
  1602 Amino acid sequence of HPV type 33 L1 protein aa 474-499
KAKPKLKRAAPTSTRTSSAKRKKVKK

SEQ ID NO: 29 - protein, 500 aa, Artificial sequence
  1603 Amino acid sequence of chimeric HPV type 16 L1 protein
MSLWLPSEATVYLPPVPVSKVVSTDEYVARTNIYYHAGTSRLLAVGHPYFPIKKPNNNKILVPKVSGLQYRVFRIHLPDPNKFGFPDTSFYNPDTQRLVWACVGVEVGRGQPLGVGISGHPLLNKLDDTENASAYAANAGVDNRECISMDYKQTQLCLIGCKPPIGEHWGKGSPCTNVAVNPGDCPPLELINTVIQDGDMVDTGFGAMDFTTLQANKSEVPLDICTSICKYPDYIKMVSEPYGDSLFFYLRREQMFVRHLFNRAGAVGENVPDDLYIKGSGSTANLASSNYFPTPSGSMVTSDAQIFNKPYWLQRAQGHNNGICWGNQLFVTVVDTTRSTNMSLCAAISTSETTYKNTNFKEYLRHGEEYDLQFIFQLCKITLTADVMTYIHSMNSTILEDWNFGLQPPPGGTLEDTYRFVTSQAIACQKHTPPAPKEDPLKKYTFWEVNLKEKFSADLDQFPLGRKFLLQAGLKAKPKLKRAAPTSTRTSSAKRKKVKK

SEQ ID NO: 30 - DNA, 1504 bp, Artificial sequence
  1604 Nucleotide sequence of chimeric HPV type 16 L1 protein
atgagtctgtggctgccatctgaggctacagtctacctgcctcctgtgcctgtgagcaaggtggtgagcacagatgaatatgtggcaaggaccaacatctactaccatgctggcaccagcagactgctggctgtgggacacccatactttccaatcaagaagccaaacaacaacaagattctggtgccaaaggtgtctggactccaatacagggtgttcaggattcacctgcctgacccaaacaagtttggctttcctgacacctccttctacaaccctgacacccagagactggtgtgggcttgtgtgggagtggaggtgggcaggggacaaccactgggagtgggcatctctggacacccactgctgaacaaactggatgacacagagaatgcctctgcctatgctgccaatgctggagtggacaacagggagtgtatcagtatggactacaagcagacccaactttgtctgattggctgtaagcctccaattggagaacactggggcaagggcagcccatgtaccaatgtggctgtgaaccctggagactgtcctccattggaactgataaacacagtgattcaggatggagatatggtggacacaggctttggagctatggacttcaccaccctccaagccaacaagtctgaggtgccactggacatctgtaccagcatctgtaaataccctgactacatcaagatggtgtctgaaccatatggagactccctgttcttctacctgaggagggaacagatgtttgtgagacacctgttcaacagggctggagcagtgggagagaatgtgcctgatgacctctacatcaagggctctggcagcacagccaacctggcatccagcaactactttccaacaccatctggcagtatggtgacctctgatgcccagattttcaacaagccatactggctccaaagggctcaaggacacaacaatggcatctgttggggcaaccaactttttgtgacagtggtggacaccaccaggagcaccaatatgagtctgtgtgctgccatcagcacctctgagaccacctacaagaacaccaacttcaaggaatacctgagacatggagaggaatatgacctccaattcatcttccaactttgtaagattaccctgacagcagatgtgatgacctacatccacagtatgaacagcaccatcttggaggactggaactttggactccaacctcctcctggaggcaccttggaggacacctacaggtttgtgaccagccaggctattgcctgtcagaaacacacacctcctgccccaaaggaggacccactgaaaaaatacaccttctgggaggtgaacctgaaagagaagttctctgctgacctggaccagtttccactgggcaggaagttcctgctccaagcaggactgaaagccaagccaaaactgaaaagggctgccccaaccagcaccaggacctcctctgccaagaggaagaaggtgaagaagtaaa

SEQ ID NO: 31 - DNA, 1537 bp, Artificial sequence
  1605 Synthetic HPV16 L1 gene
ctgggtaccatgagtctgtggctgccatctgaggctacagtctacctgcctcctgtgcctgtgagcaaggtggtgagcacagatgaatatgtggcaaggaccaacatctactaccatgctggcaccagcagactgctggctgtgggacacccatactttccaatcaagaagccaaacaacaacaagattctggtgccaaaggtgtctggactccaatacagggtgttcaggattcacctgcctgacccaaacaagtttggctttcctgacacctccttctacaaccctgacacccagagactggtgtgggcttgtgtgggagtggaggtgggcaggggacaaccactgggagtgggcatctctggacacccactgctgaacaaactggatgacacagagaatgcctctgcctatgctgccaatgctggagtggacaacagggagtgtatcagtatggactacaagcagacccaactttgtctgattggctgtaagcctccaattggagaacactggggcaagggcagcccatgtaccaatgtggctgtgaaccctggagactgtcctccattggaactgataaacacagtgattcaggatggagatatggtggacacaggctttggagctatggacttcaccaccctccaagccaacaagtctgaggtgccactggacatctgtaccagcatctgtaaataccctgactacatcaagatggtgtctgaaccatatggagactccctgttcttctacctgaggagggaacagatgtttgtgagacacctgttcaacagggctggagcagtgggagagaatgtgcctgatgacctctacatcaagggctctggcagcacagccaacctggcatccagcaactactttccaacaccatctggcagtatggtgacctctgatgcccagattttcaacaagccatactggctccaaagggctcaaggacacaacaatggcatctgttggggcaaccaactttttgtgacagtggtggacaccaccaggagcaccaatatgagtctgtgtgctgccatcagcacctctgagaccacctacaagaacaccaacttcaaggaatacctgagacatggagaggaatatgacctccaattcatcttccaactttgtaagattaccctgacagcagatgtgatgacctacatccacagtatgaacagcaccatcttggaggactggaactttggactccaacctcctcctggaggcaccttggaggacacctacaggtttgtgaccagccaggctattgcctgtcagaaacacacacctcctgccccaaaggaggacccactgaaaaaatacaccttctgggaggtgaacctgaaagagaagttctctgctgacctggaccagtttccactgggcaggaagttcctgctccaagcaggactgaaagccaagccaaagttcaccctgggcaagaggaaggctacaccaaccacctccagcaccagcaccacagccaagaggaagaagaggaaactgtaaactcgagctc

SEQ ID NO: 32 - DNA, 1519 bp, Artificial sequence; identical to SEQ ID NO: 6
  1606 Synthetic HPV33 L1 gene

SEQ ID NO: 33 - DNA, 34 bp, Artificial sequence
  1607 HPV16L1 F1
cttggtaccatgagtctgtggctgccatctgagg

SEQ ID NO: 34 - DNA, 36 bp, Artificial sequence
  1608 HPV16L1 R1
gcttggctttcagtcctgcttggagcaggaacttcc

SEQ ID NO: 35 - DNA, 1441 bp, Artificial sequence
  1609 HPV16L1 amplified sequence 1
cttggtaccatgagtctgtggctgccatctgaggctacagtctacctgcctcctgtgcctgtgagcaaggtggtgagcacagatgaatatgtggcaaggaccaacatctactaccatgctggcaccagcagactgctggctgtgggacacccatactttccaatcaagaagccaaacaacaacaagattctggtgccaaaggtgtctggactccaatacagggtgttcaggattcacctgcctgacccaaacaagtttggctttcctgacacctccttctacaaccctgacacccagagactggtgtgggcttgtgtgggagtggaggtgggcaggggacaaccactgggagtgggcatctctggacacccactgctgaacaaactggatgacacagagaatgcctctgcctatgctgccaatgctggagtggacaacagggagtgtatcagtatggactacaagcagacccaactttgtctgattggctgtaagcctccaattggagaacactggggcaagggcagcccatgtaccaatgtggctgtgaaccctggagactgtcctccattggaactgataaacacagtgattcaggatggagatatggtggacacaggctttggagctatggacttcaccaccctccaagccaacaagtctgaggtgccactggacatctgtaccagcatctgtaaataccctgactacatcaagatggtgtctgaaccatatggagactccctgttcttctacctgaggagggaacagatgtttgtgagacacctgttcaacagggctggagcagtgggagagaatgtgcctgatgacctctacatcaagggctctggcagcacagccaacctggcatccagcaactactttccaacaccatctggcagtatggtgacctctgatgcccagattttcaacaagccatactggctccaaagggctcaaggacacaacaatggcatctgttggggcaaccaactttttgtgacagtggtggacaccaccaggagcaccaatatgagtctgtgtgctgccatcagcacctctgagaccacctacaagaacaccaacttcaaggaatacctgagacatggagaggaatatgacctccaattcatcttccaactttgtaagattaccctgacagcagatgtgatgacctacatccacagtatgaacagcaccatcttggaggactggaactttggactccaacctcctcctggaggcaccttggaggacacctacaggtttgtgaccagccaggctattgcctgtcagaaacacacacctcctgccccaaaggaggacccactgaaaaaatacaccttctgggaggtgaacctgaaagagaagttctctgctgacctggaccagtttccactgggcaggaagttcctgctccaagcaggactgaaagccaagc

SEQ ID NO: 36 - DNA, 35 bp, Artificial sequence
  1610 HPV16L1 F2
agcaggactgaaagccaagccaaaactgaaaaggg

SEQ ID NO: 37 - DNA, 36 bp, Artificial sequence
  1611 HPV16L1 R2
ctgtctagatttacttcttcaccttcttcctcttgg

SEQ ID NO: 38 - DNA, 101 bp, Artificial sequence
  1612 HPV16L1 amplified sequence 2
agcaggactgaaagccaagccaaaactgaaaagggctgccccaaccagcaccaggacctcctctgccaagaggaagaaggtgaagaagtaaatctagacag

SEQ ID NO: 39 - protein, 38 aa, Homo sapiens; identical to SEQ ID NO: 13
  1613 Amino acid sequence of HPV type 59 L1 protein aa 471-508

SEQ ID NO: 40 - protein, 470 aa, Homo sapiens
  1801 Amino acid sequence of HPV type 18 L1 protein aa 1-470
MALWRPSDNTVYLPPPSVARVVNTDDYVTRTSIFYHAGSSRLLTVGNPYFRVPAGGGNKQDIPKVSAYQYRVFRVQLPDPNKFGLPDTSIYNPETQRLVWACAGVEIGRGQPLGVGLSGHPFYNKLDDTESSHAATSNVSEDVRDNVSVDYKQTQLCILGCAPAIGEHWAKGTACKSRPLSQGDCPPLELKNTVLEDGDMVDTGYGAMDFSTLQDTKCEVPLDICQSICKYPDYLQMSADPYGDSMFFCLRREQLFARHFWNRAGTMGDTVPQSLYIKGTGMRASPGSCVYSPSPSGSIVTSDSQLFNKPYWLHKAQGHNNGVCWHNQLFVTVVDTTRSTNLTICASTQSPVPGQYDATKFKQYSRHVEEYDLQFIFQLCTITLTADVMSYIHSMNSSILEDWNFGVPPPPTTSLVDTYRFVQSVAITCQKDAAPAENKDPYDKLKFWNVDLKEKFSLDLDQYPLGRKFL

SEQ ID NO: 41 - protein, 26 aa, Homo sapiens
  1802 Amino acid sequence of HPV type 33 L1 protein aa 474-499
KAKPKLKRAAPTSTRTSSAKRKKVKK

SEQ ID NO: 42 - protein, 496 aa, Artificial sequence
  1803 Amino acid sequence of chimeric HPV type 18 L1 protein
MALWRPSDNTVYLPPPSVARVVNTDDYVTRTSIFYHAGSSRLLTVGNPYFRVPAGGGNKQDIPKVSAYQYRVFRVQLPDPNKFGLPDTSIYNPETQRLVWACAGVEIGRGQPLGVGLSGHPFYNKLDDTESSHAATSNVSEDVRDNVSVDYKQTQLCILGCAPAIGEHWAKGTACKSRPLSQGDCPPLELKNTVLEDGDMVDTGYGAMDFSTLQDTKCEVPLDICQSICKYPDYLQMSADPYGDSMFFCLRREQLFARHFWNRAGTMGDTVPQSLYIKGTGMRASPGSCVYSPSPSGSIVTSDSQLFNKPYWLHKAQGHNNGVCWHNQLFVTVVDTTRSTNLTICASTQSPVPGQYDATKFKQYSRHVEEYDLQFIFQLCTITLTADVMSYIHSMNSSILEDWNFGVPPPPTTSLVDTYRFVQSVAITCQKDAAPAENKDPYDKLKFWNVDLKEKFSLDLDQYPLGRKFLKAKPKLKRAAPTSTRTSSAKRKKVKK

SEQ ID NO: 43 - DNA, 1492 bp, Artificial sequence
  1804 Nucleotide sequence of chimeric HPV type 18 L1 protein
atggccctctggagaccatccgataacacagtgtacttgcccccacccagcgtcgcccgggtggtgaacacagacgactacgtcaccagaacctcaatcttctaccacgccgggtccagccggctgctgaccgtgggcaacccctacttccgcgtgcccgccggcggcggaaacaaacaagacatccccaaagtcagcgcctatcagtaccgggtgttccgcgtccaactgcccgatcccaacaagttcggcctgcccgacacctccatctacaaccccgagacccagaggctggtctgggcttgcgccggcgtcgagatcgggaggggccaacccctgggcgtggggttgtccggccaccccttctacaacaagctggacgataccgagtccagccacgcagcaaccagcaacgtctccgaagatgtgcgcgataacgtcagcgtggactacaaacaaacccaactgtgcatcctgggatgcgcacccgccatcggcgagcattgggccaaggggaccgcctgcaagagcaggcccctgagccaaggggactgtccacccctggagttgaagaataccgtgctcgaggacggcgacatggtggacaccggctacggcgctatggatttctccaccctccaggacaccaagtgcgaagtgcccctcgacatctgccaaagcatctgcaagtaccccgactacctccagatgagcgccgacccctacggcgacagcatgttcttctgtctcagaagggaacaattgttcgcccgccacttctggaaccgggccggcacaatgggagatacagtcccccagagcctgtacatcaaggggaccggaatgagggccagccccgggtcctgcgtctacagcccaagcccctccgggagcatcgtcacaagcgatagccaactcttcaacaagccctactggctccacaaagcccaaggccacaataacggggtgtgttggcacaaccagctgttcgtgaccgtcgtggacacaaccaggtccacaaacctgaccatctgcgccagcacccaaagccccgtgcccggccagtacgacgccacaaagttcaaacaatactctcggcacgtggaagagtacgacctccaattcatcttccaactctgcaccatcaccctcaccgccgacgtgatgagctacatccactccatgaactcctccatcctggaagactggaatttcggcgtgccaccaccccctaccacctccctcgtcgacacctacagattcgtgcagagcgtggccatcacatgccagaaagacgccgcccccgccgagaacaaagacccatacgacaaactgaaattctggaacgtcgacctgaaagagaaattcagcctggatctggaccagtacccattgggcaggaagttcctcaaagccaagccaaaactgaaaagggctgccccaaccagcaccaggacctcctctgccaagaggaagaaggtgaagaagtaaa

SEQ ID NO: 44 - DNA, 1543 bp, Artificial sequence
  1805 Synthetic HPV18 L1 gene
ctgggtaccatggccctctggagaccatccgataacacagtgtacttgcccccacccagcgtcgcccgggtggtgaacacagacgactacgtcaccagaacctcaatcttctaccacgccgggtccagccggctgctgaccgtgggcaacccctacttccgcgtgcccgccggcggcggaaacaaacaagacatccccaaagtcagcgcctatcagtaccgggtgttccgcgtccaactgcccgatcccaacaagttcggcctgcccgacacctccatctacaaccccgagacccagaggctggtctgggcttgcgccggcgtcgagatcgggaggggccaacccctgggcgtggggttgtccggccaccccttctacaacaagctggacgataccgagtccagccacgcagcaaccagcaacgtctccgaagatgtgcgcgataacgtcagcgtggactacaaacaaacccaactgtgcatcctgggatgcgcacccgccatcggcgagcattgggccaaggggaccgcctgcaagagcaggcccctgagccaaggggactgtccacccctggagttgaagaataccgtgctcgaggacggcgacatggtggacaccggctacggcgctatggatttctccaccctccaggacaccaagtgcgaagtgcccctcgacatctgccaaagcatctgcaagtaccccgactacctccagatgagcgccgacccctacggcgacagcatgttcttctgtctcagaagggaacaattgttcgcccgccacttctggaaccgggccggcacaatgggagatacagtcccccagagcctgtacatcaaggggaccggaatgagggccagccccgggtcctgcgtctacagcccaagcccctccgggagcatcgtcacaagcgatagccaactcttcaacaagccctactggctccacaaagcccaaggccacaataacggggtgtgttggcacaaccagctgttcgtgaccgtcgtggacacaaccaggtccacaaacctgaccatctgcgccagcacccaaagccccgtgcccggccagtacgacgccacaaagttcaaacaatactctcggcacgtggaagagtacgacctccaattcatcttccaactctgcaccatcaccctcaccgccgacgtgatgagctacatccactccatgaactcctccatcctggaagactggaatttcggcgtgccaccaccccctaccacctccctcgtcgacacctacagattcgtgcagagcgtggccatcacatgccagaaagacgccgcccccgccgagaacaaagacccatacgacaaactgaaattctggaacgtcgacctgaaagagaaattcagcctggatctggaccagtacccattgggcaggaagttcctcgtgcaagccggcctcaggagaaaaccaacaatcgggcccaggaagaggagcgcccccagcgcaaccaccagcagcaagcccgcaaaaagggtcagagtgagggcacgcaaataaactcgagctc

SEQ ID NO: 45 - DNA, 1519 bp, Artificial sequence; identical to SEQ ID NO: 6
  1806 Synthetic HPV33 L1 gene

SEQ ID NO: 46 - DNA, 34 bp, Artificial sequence
  1807 HPV18L1 F1
cttggtaccatggccctctggagaccatccgata

SEQ ID NO: 47 - DNA, 35 bp, Artificial sequence
  1808 HPV18L1 R1
gcttggctttgaggaacttcctgcccaatgggtac

SEQ ID NO: 48 - DNA, 1429 bp, Artificial sequence
  1809 HPV18L1 amplified sequence 1
cttggtaccatggccctctggagaccatccgataacacagtgtacttgcccccacccagcgtcgcccgggtggtgaacacagacgactacgtcaccagaacctcaatcttctaccacgccgggtccagccggctgctgaccgtgggcaacccctacttccgcgtgcccgccggcggcggaaacaaacaagacatccccaaagtcagcgcctatcagtaccgggtgttccgcgtccaactgcccgatcccaacaagttcggcctgcccgacacctccatctacaaccccgagacccagaggctggtctgggcttgcgccggcgtcgagatcgggaggggccaacccctgggcgtggggttgtccggccaccccttctacaacaagctggacgataccgagtccagccacgcagcaaccagcaacgtctccgaagatgtgcgcgataacgtcagcgtggactacaaacaaacccaactgtgcatcctgggatgcgcacccgccatcggcgagcattgggccaaggggaccgcctgcaagagcaggcccctgagccaaggggactgtccacccctggagttgaagaataccgtgctcgaggacggcgacatggtggacaccggctacggcgctatggatttctccaccctccaggacaccaagtgcgaagtgcccctcgacatctgccaaagcatctgcaagtaccccgactacctccagatgagcgccgacccctacggcgacagcatgttcttctgtctcagaagggaacaattgttcgcccgccacttctggaaccgggccggcacaatgggagatacagtcccccagagcctgtacatcaaggggaccggaatgagggccagccccgggtcctgcgtctacagcccaagcccctccgggagcatcgtcacaagcgatagccaactcttcaacaagccctactggctccacaaagcccaaggccacaataacggggtgtgttggcacaaccagctgttcgtgaccgtcgtggacacaaccaggtccacaaacctgaccatctgcgccagcacccaaagccccgtgcccggccagtacgacgccacaaagttcaaacaatactctcggcacgtggaagagtacgacctccaattcatcttccaactctgcaccatcaccctcaccgccgacgtgatgagctacatccactccatgaactcctccatcctggaagactggaatttcggcgtgccaccaccccctaccacctccctcgtcgacacctacagattcgtgcagagcgtggccatcacatgccagaaagacgccgcccccgccgagaacaaagacccatacgacaaactgaaattctggaacgtcgacctgaaagagaaattcagcctggatctggaccagtacccattgggcaggaagttcctcaaagccaagc

SEQ ID NO: 49 - DNA, 35 bp, Artificial sequence
  1810 HPV18L1 F2
gaagttcctcaaagccaagccaaaactgaaaaggg

SEQ ID NO: 50 - DNA, 36 bp, Artificial sequence; identical to SEQ ID NO: 37
  1811 HPV18L1 R2

SEQ ID NO: 51 - DNA, 101 bp, Artificial sequence
  1812 HPV18L1 amplified sequence 2
gaagttcctcaaagccaagccaaaactgaaaagggctgccccaaccagcaccaggacctcctctgccaagaggaagaaggtgaagaagtaaatctagacag

SEQ ID NO: 52 - protein, 38 aa, Homo sapiens; identical to SEQ ID NO: 13
  1813 Amino acid sequence of HPV type 59 L1 protein aa 471-508

SEQ ID NO: 53 - protein, 475 aa, Homo sapiens
  3101 Amino acid sequence of HPV type 31 L1 protein aa 1-475
MSLWRPSEATVYLPPVPVSKVVSTDEYVTRTNIYYHAGSARLLTVGHPYYSIPKSDNPKKIVVPKVSGLQYRVFRVRLPDPNKFGFPDTSFYNPETQRLVWACVGLEVGRGQPLGVGISGHPLLNKFDDTENSNRYAGGPGTDNRECISMDYKQTQLCLLGCKPPIGEHWGKGSPCSNNAITPGDCPPLELKNSVIQDGDMVDTGFGAMDFTALQDTKSNVPLDICNSICKYPDYLKMVAEPYGDTLFFYLRREQMFVRHFFNRSGTVGESVPTDLYIKGSGSTATLANSTYFPTPSGSMVTSDAQIFNKPYWMQRAQGHNNGICWGNQLFVTVVDTTRSTNMSVCAAIANSDTTFKSSNFKEYLRHGEEFDLQFIFQLCKITLSADIMTYIHSMNPAILEDWNFGLTTPPSGSLEDTYRFVTSQAITCQKSAPQKPKEDPFKDYVFWEVNLKEKFSADLDQFPLGRKFLLQAGY

SEQ ID NO: 54 - protein, 26 aa, Homo sapiens
  3102 Amino acid sequence of HPV type 33 L1 protein aa 474-499
KAKPKLKRAAPTSTRTSSAKRKKVKK

SEQ ID NO: 55 - protein, 501 aa, Artificial sequence
  3103 Amino acid sequence of chimeric HPV type 31 L1 protein
MSLWRPSEATVYLPPVPVSKVVSTDEYVTRTNIYYHAGSARLLTVGHPYYSIPKSDNPKKIVVPKVSGLQYRVFRVRLPDPNKFGFPDTSFYNPETQRLVWACVGLEVGRGQPLGVGISGHPLLNKFDDTENSNRYAGGPGTDNRECISMDYKQTQLCLLGCKPPIGEHWGKGSPCSNNAITPGDCPPLELKNSVIQDGDMVDTGFGAMDFTALQDTKSNVPLDICNSICKYPDYLKMVAEPYGDTLFFYLRREQMFVRHFFNRSGTVGESVPTDLYIKGSGSTATLANSTYFPTPSGSMVTSDAQIFNKPYWMQRAQGHNNGICWGNQLFVTVVDTTRSTNMSVCAAIANSDTTFKSSNFKEYLRHGEEFDLQFIFQLCKITLSADIMTYIHSMNPAILEDWNFGLTTPPSGSLEDTYRFVTSQAITCQKSAPQKPKEDPFKDYVFWEVNLKEKFSADLDQFPLGRKFLLQAGYKAKPKLKRAAPTSTRTSSAKRKKVKK

SEQ ID NO: 56 - DNA, 1507 bp, Artificial sequence
  3104 Nucleotide sequence of chimeric HPV type 31 L1 protein
atgagcctgtggaggcccagcgaggccaccgtgtacctgccccccgtgcccgtgagcaaggtggtgagcaccgacgagtacgtgaccaggaccaacatctactaccacgccggcagcgccaggctgctgaccgtgggccacccctactacagcatccccaagagcgacaaccccaagaagatcgtggtgcccaaggtgagcggcctgcagtacagggtgttcagggtgaggctgcccgaccccaacaagttcggcttccccgacaccagcttctacaaccccgagacccagaggctggtgtgggcctgcgtgggcctggaggtgggcaggggccagcccctgggcgtgggcatcagcggccaccccctgctgaacaagttcgacgacaccgagaacagcaacaggtacgccggcggccccggcaccgacaacagggagtgcatcagcatggactacaagcagacccagctgtgcctgctgggctgcaagccccccatcggcgagcactggggcaagggcagcccctgcagcaacaacgccatcacccccggcgactgcccccccctggagctgaagaacagcgtgatccaggacggcgacatggtggacaccggcttcggcgccatggacttcaccgccctgcaggacaccaagagcaacgtgcccctggacatctgcaacagcatctgcaagtaccccgactacctgaagatggtggccgagccctacggcgacaccctgttcttctacctgaggagggagcagatgttcgtgaggcacttcttcaacaggagcggcaccgtgggcgagagcgtgcccaccgacctgtacatcaagggcagcggcagcaccgccaccctggccaacagcacctacttccccacccccagcggcagcatggtgaccagcgacgcccagatcttcaacaagccctactggatgcagagggcccagggccacaacaacggcatctgctggggcaaccagctgttcgtgaccgtggtggacaccaccaggagcaccaacatgagcgtgtgcgccgccatcgccaacagcgacaccaccttcaagagcagcaacttcaaggagtacctgaggcacggcgaggagttcgacctgcagttcatcttccagctgtgcaagatcaccctgagcgccgacatcatgacctacatccacagcatgaaccccgccatcctggaggactggaacttcggcctgaccaccccccccagcggcagcctggaggacacctacaggttcgtgaccagccaggccatcacctgccagaagtccgccccccagaagcccaaggaggaccccttcaaggactacgtgttctgggaggtgaacctgaaggagaagttcagcgccgacctggaccagttccccctgggcaggaagttcctgctgcaggccggctacaaagccaagccaaaactgaaaagggctgccccaaccagcaccaggacctcctctgccaagaggaagaaggtgaagaagtaaa

SEQ ID NO: 57 - DNA, 1534 bp, Artificial sequence
  3105 Synthetic HPV31 L1 gene
ctgggtaccatgagcctgtggaggcccagcgaggccaccgtgtacctgccccccgtgcccgtgagcaaggtggtgagcaccgacgagtacgtgaccaggaccaacatctactaccacgccggcagcgccaggctgctgaccgtgggccacccctactacagcatccccaagagcgacaaccccaagaagatcgtggtgcccaaggtgagcggcctgcagtacagggtgttcagggtgaggctgcccgaccccaacaagttcggcttccccgacaccagcttctacaaccccgagacccagaggctggtgtgggcctgcgtgggcctggaggtgggcaggggccagcccctgggcgtgggcatcagcggccaccccctgctgaacaagttcgacgacaccgagaacagcaacaggtacgccggcggccccggcaccgacaacagggagtgcatcagcatggactacaagcagacccagctgtgcctgctgggctgcaagccccccatcggcgagcactggggcaagggcagcccctgcagcaacaacgccatcacccccggcgactgcccccccctggagctgaagaacagcgtgatccaggacggcgacatggtggacaccggcttcggcgccatggacttcaccgccctgcaggacaccaagagcaacgtgcccctggacatctgcaacagcatctgcaagtaccccgactacctgaagatggtggccgagccctacggcgacaccctgttcttctacctgaggagggagcagatgttcgtgaggcacttcttcaacaggagcggcaccgtgggcgagagcgtgcccaccgacctgtacatcaagggcagcggcagcaccgccaccctggccaacagcacctacttccccacccccagcggcagcatggtgaccagcgacgcccagatcttcaacaagccctactggatgcagagggcccagggccacaacaacggcatctgctggggcaaccagctgttcgtgaccgtggtggacaccaccaggagcaccaacatgagcgtgtgcgccgccatcgccaacagcgacaccaccttcaagagcagcaacttcaaggagtacctgaggcacggcgaggagttcgacctgcagttcatcttccagctgtgcaagatcaccctgagcgccgacatcatgacctacatccacagcatgaaccccgccatcctggaggactggaacttcggcctgaccaccccccccagcggcagcctggaggacacctacaggttcgtgaccagccaggccatcacctgccagaagtccgccccccagaagcccaaggaggaccccttcaaggactacgtgttctgggaggtgaacctgaaggagaagttcagcgccgacctggaccagttccccctgggcaggaagttcctgctgcaggccggctacagggccaggcccaagttcaaggccggcaagaggagcgcccccagcgccagcaccaccacccccgccaagaggaagaagaccaagaagtaaactcgagctc

SEQ ID NO: 58 - DNA, 1519 bp, Artificial sequence; identical to SEQ ID NO: 6
  3106 Synthetic HPV33 L1 gene

SEQ ID NO: 59 - DNA, 33 bp, Artificial sequence
  3107 HPV31L1 F1
cttggtaccatgagcctgtggaggcccagcgag

SEQ ID NO: 60 - DNA, 38 bp, Artificial sequence
  3108 HPV31L1 R1
gcttggctttgtagccggcctgcagcaggaacttcctg

SEQ ID NO: 61 - DNA, 1444 bp, Artificial sequence
  3109 HPV31L1 amplified sequence 1
cttggtaccatgagcctgtggaggcccagcgaggccaccgtgtacctgccccccgtgcccgtgagcaaggtggtgagcaccgacgagtacgtgaccaggaccaacatctactaccacgccggcagcgccaggctgctgaccgtgggccacccctactacagcatccccaagagcgacaaccccaagaagatcgtggtgcccaaggtgagcggcctgcagtacagggtgttcagggtgaggctgcccgaccccaacaagttcggcttccccgacaccagcttctacaaccccgagacccagaggctggtgtgggcctgcgtgggcctggaggtgggcaggggccagcccctgggcgtgggcatcagcggccaccccctgctgaacaagttcgacgacaccgagaacagcaacaggtacgccggcggccccggcaccgacaacagggagtgcatcagcatggactacaagcagacccagctgtgcctgctgggctgcaagccccccatcggcgagcactggggcaagggcagcccctgcagcaacaacgccatcacccccggcgactgcccccccctggagctgaagaacagcgtgatccaggacggcgacatggtggacaccggcttcggcgccatggacttcaccgccctgcaggacaccaagagcaacgtgcccctggacatctgcaacagcatctgcaagtaccccgactacctgaagatggtggccgagccctacggcgacaccctgttcttctacctgaggagggagcagatgttcgtgaggcacttcttcaacaggagcggcaccgtgggcgagagcgtgcccaccgacctgtacatcaagggcagcggcagcaccgccaccctggccaacagcacctacttccccacccccagcggcagcatggtgaccagcgacgcccagatcttcaacaagccctactggatgcagagggcccagggccacaacaacggcatctgctggggcaaccagctgttcgtgaccgtggtggacaccaccaggagcaccaacatgagcgtgtgcgccgccatcgccaacagcgacaccaccttcaagagcagcaacttcaaggagtacctgaggcacggcgaggagttcgacctgcagttcatcttccagctgtgcaagatcaccctgagcgccgacatcatgacctacatccacagcatgaaccccgccatcctggaggactggaacttcggcctgaccaccccccccagcggcagcctggaggacacctacaggttcgtgaccagccaggccatcacctgccagaagtccgccccccagaagcccaaggaggaccccttcaaggactacgtgttctgggaggtgaacctgaaggagaagttcagcgccgacctggaccagttccccctgggcaggaagttcctgctgcaggccggctacaaagccaagc

SEQ ID NO: 62 - DNA, 35 bp, Artificial sequence
  3110 HPV31L1 F2
ggccggctacaaagccaagccaaaactgaaaaggg

SEQ ID NO: 63 - DNA, 41 bp, Artificial sequence
  3111 HPV31L1 R2
ctgtctagatttacttcttcaccttcttcctcttggcagag

SEQ ID NO: 64 - DNA, 101 bp, Artificial sequence
  3112 HPV31L1 amplified sequence 2
ggccggctacaaagccaagccaaaactgaaaagggctgccccaaccagcaccaggacctcctctgccaagaggaagaaggtgaagaagtaaatctagacag

SEQ ID NO: 65 - protein, 38 aa, Homo sapiens; identical to SEQ ID NO: 13
  3113 Amino acid sequence of HPV type 59 L1 protein aa 471-508

SEQ ID NO: 66 - protein, 499 aa, Homo sapiens
  3301 Amino acid sequence of HPV type 33 L1 protein
MSVWRPSEATVYLPPVPVSKVVSTDEYVSRTSIYYYAGSSRLLAVGHPYFSIKNPTNAKKLLVPKVSGLQYRVFRVRLPDPNKFGFPDTSFYNPDTQRLVWACVGLEIGRGQPLGVGISGHPLLNKFDDTETGNKYPGQPGADNRECLSMDYKQTQLCLLGCKPPTGEHWGKGVACTNAAPANDCPPLELINTIIEDGDMVDTGFGCMDFKTLQANKSDVPIDICGSTCKYPDYLKMTSEPYGDSLFFFLRREQMFVRHFFNRAGTLGEAVPDDLYIKGSGTTASIQSSAFFPTPSGSMVTSESQLFNKPYWLQRAQGHNNGICWGNQVFVTVVDTTRSTNMTLCTQVTSDSTYKNENFKEYIRHVEEYDLQFVFQLCKVTLTAEVMTYIHAMNPDILEDWQFGLTPPPSASLQDTYRFVTSQAITCQKTVPPKEKEDPLGKYTFWEVDLKEKFSADLDQFPLGRKFLLQAGLKAKPKLKRAAPTSTRTSSAKRKKVKK

SEQ ID NO: 67 - DNA, 1501 bp, Homo sapiens
  3302 Nucleotide sequence of HPV type 33 L1 protein
atgagtgtgtggagaccatctgaggctacagtctacctgcctcctgtgcctgtgagcaaggtggtgagcacagatgaatatgtgagcaggaccagcatctactactatgctggctccagcagactgctggctgtgggacacccatacttcagcatcaagaacccaaccaatgccaagaaactgctggtgccaaaggtgtctggactccaatacagggtgttcagggtgagactgcctgacccaaacaagtttggctttcctgacacctccttctacaaccctgacacccagagactggtgtgggcttgtgtgggattggagattggcaggggacaaccactgggagtgggcatctctggacacccactgctgaacaagtttgatgacacagagacaggcaacaaataccctggacaacctggagcagacaacagggagtgtctgagtatggactacaagcagacccaactttgtctgctgggctgtaagcctccaacaggagaacactggggcaagggagtggcttgtaccaatgctgcccctgccaatgactgtcctccattggaactgataaacaccatcattgaggatggagatatggtggacacaggctttggctgtatggacttcaagaccctccaagccaacaagtctgatgtgccaattgacatctgtggcagcacttgtaaataccctgactacctgaaaatgacctctgaaccatatggagactccctgttcttcttcctgaggagggaacagatgtttgtgagacacttcttcaacagggctggcaccctgggagaggctgtgcctgatgacctctacatcaagggctctggcaccacagccagcatccagtcctctgccttctttccaacaccatctggcagtatggtgacctctgagagccaacttttcaacaagccatactggctccaaagggctcaaggacacaacaatggcatctgttggggcaaccaggtgtttgtgacagtggtggacaccaccaggagcaccaatatgaccctgtgtacccaggtgacctctgacagcacctacaagaatgagaacttcaaggaatacatcaggcatgtggaggaatatgacctccaatttgtgttccaactttgtaaggtgaccctgacagcagaggtgatgacctacatccatgctatgaaccctgacatcttggaggactggcagtttggactgacacctcctccatctgcctccctccaagacacctacaggtttgtgaccagccaggctatcacttgtcagaagacagtgcctccaaaggagaaggaggacccactgggcaaatacaccttctgggaggtggacctgaaagagaagttctctgctgacctggaccagtttccactgggcaggaagttcctgctccaagcaggactgaaagccaagccaaaactgaaaagggctgccccaaccagcaccaggacctcctctgccaagaggaagaaggtgaagaagtaaa

SEQ ID NO: 68 - DNA, 1519 bp, Artificial sequence; identical to SEQ ID NO: 6
  3303 Synthetic HPV33 L1 gene

SEQ ID NO: 69 - protein, 472 aa, Homo sapiens
  3501 Amino acid sequence of HPV type 35 L1 protein aa 1-472
MSLWRSNEATVYLPPVSVSKVVSTDEYVTRTNIYYHAGSSRLLAVGHPYYAIKKQDSNKIAVPKVSGLQYRVFRVKLPDPNKFGFPDTSFYDPASQRLVWACTGVEVGRGQPLGVGISGHPLLNKLDDTENSNKYVGNSGTDNRECISMDYKQTQLCLIGCRPPIGEHWGKGTPCNANQVKAGECPPLELLNTVLQDGDMVDTGFGAMDFTTLQANKSDVPLDICSSICKYPDYLKMVSEPYGDMLFFYLRREQMFVRHLFNRAGTVGETVPADLYIKGTTGTLPSTSYFPTPSGSMVTSDAQIFNKPYWLQRAQGHNNGICWSNQLFVTVVDTTRSTNMSVCSAVSSSDSTYKNDNFKEYLRHGEEYDLQFIFQLCKITLTADVMTYIHSMNPSILEDWNFGLTPPPSGTLEDTYRYVTSQAVTCQKPSAPKPKDDPLKNYTFWEVDLKEKFSADLDQFPLGRKFLLQAGL

SEQ ID NO: 70 - protein, 26 aa, Homo sapiens
  3502 Amino acid sequence of HPV type 33 L1 protein aa 474-499
KAKPKLKRAAPTSTRTSSAKRKKVKK

SEQ ID NO: 71 - protein, 498 aa, Artificial sequence
  3503 Amino acid sequence of chimeric HPV type 35 L1 protein
MSLWRSNEATVYLPPVSVSKVVSTDEYVTRTNIYYHAGSSRLLAVGHPYYAIKKQDSNKIAVPKVSGLQYRVFRVKLPDPNKFGFPDTSFYDPASQRLVWACTGVEVGRGQPLGVGISGHPLLNKLDDTENSNKYVGNSGTDNRECISMDYKQTQLCLIGCRPPIGEHWGKGTPCNANQVKAGECPPLELLNTVLQDGDMVDTGFGAMDFTTLQANKSDVPLDICSSICKYPDYLKMVSEPYGDMLFFYLRREQMFVRHLFNRAGTVGETVPADLYIKGTTGTLPSTSYFPTPSGSMVTSDAQIFNKPYWLQRAQGHNNGICWSNQLFVTVVDTTRSTNMSVCSAVSSSDSTYKNDNFKEYLRHGEEYDLQFIFQLCKITLTADVMTYIHSMNPSILEDWNFGLTPPPSGTLEDTYRYVTSQAVTCQKPSAPKPKDDPLKNYTFWEVDLKEKFSADLDQFPLGRKFLLQAGLKAKPKLKRAAPTSTRTSSAKRKKVKK

SEQ ID NO: 72 - DNA, 1498 bp, Artificial sequence
  3504 Nucleotide sequence of chimeric HPV type 35 L1 protein
atgagtctgtggaggagcaatgaggctacagtctacctgcctcctgtgtctgtgagcaaggtggtgagcacagatgaatatgtgaccaggaccaacatctactaccatgctggctccagcagactgctggctgtgggacacccatactatgccatcaagaagcaggacagcaacaagattgctgtgccaaaggtgtctggactccaatacagggtgttcagggtgaaactgcctgacccaaacaagtttggctttcctgacacctccttctatgaccctgccagccagagactggtgtgggcttgtactggagtggaggtgggcaggggacaaccactgggagtgggcatctctggacacccactgctgaacaaactggatgacacagagaacagcaacaaatatgtgggcaactctggcacagacaacagggagtgtatcagtatggactacaagcagacccaactttgtctgattggctgtagacctccaattggagaacactggggcaagggcacaccatgtaatgccaaccaggtgaaggctggagagtgtcctccattggaactgctgaacacagtgctccaagatggagatatggtggacacaggctttggagctatggacttcaccaccctccaagccaacaagtctgatgtgccactggacatctgttccagcatctgtaaataccctgactacctgaaaatggtgtctgaaccatatggagatatgctgttcttctacctgaggagggaacagatgtttgtgagacacctgttcaacagggctggcacagtgggagagacagtgcctgctgacctctacatcaagggcaccacaggcaccctgccaagcacctcctactttccaacaccatctggcagtatggtgacctctgatgcccagattttcaacaagccatactggctccaaagggctcaaggacacaacaatggcatctgttggagcaaccaactttttgtgacagtggtggacaccaccaggagcaccaatatgagtgtgtgttctgctgtgtcctcctctgacagcacctacaagaatgacaacttcaaggaatacctgagacatggagaggaatatgacctccaattcatcttccaactttgtaagattaccctgacagcagatgtgatgacctacatccacagtatgaacccaagcatcttggaggactggaactttggactgacacctcctccatctggcaccttggaggacacctacagatatgtgaccagccaggctgtgacttgtcagaagccatctgccccaaagccaaaggatgacccactgaaaaactacaccttctgggaggtggacctgaaagagaagttctctgctgacctggaccagtttccactgggcaggaagttcctgctccaagcaggactgaaagccaagccaaaactgaaaagggctgccccaaccagcaccaggacctcctctgccaagaggaagaaggtgaagaagtaaa

SEQ ID NO: 73 - DNA, 1528 bp, Artificial sequence
  3505 Synthetic HPV35 L1 gene
ctgggtaccatgagtctgtggaggagcaatgaggctacagtctacctgcctcctgtgtctgtgagcaaggtggtgagcacagatgaatatgtgaccaggaccaacatctactaccatgctggctccagcagactgctggctgtgggacacccatactatgccatcaagaagcaggacagcaacaagattgctgtgccaaaggtgtctggactccaatacagggtgttcagggtgaaactgcctgacccaaacaagtttggctttcctgacacctccttctatgaccctgccagccagagactggtgtgggcttgtactggagtggaggtgggcaggggacaaccactgggagtgggcatctctggacacccactgctgaacaaactggatgacacagagaacagcaacaaatatgtgggcaactctggcacagacaacagggagtgtatcagtatggactacaagcagacccaactttgtctgattggctgtagacctccaattggagaacactggggcaagggcacaccatgtaatgccaaccaggtgaaggctggagagtgtcctccattggaactgctgaacacagtgctccaagatggagatatggtggacacaggctttggagctatggacttcaccaccctccaagccaacaagtctgatgtgccactggacatctgttccagcatctgtaaataccctgactacctgaaaatggtgtctgaaccatatggagatatgctgttcttctacctgaggagggaacagatgtttgtgagacacctgttcaacagggctggcacagtgggagagacagtgcctgctgacctctacatcaagggcaccacaggcaccctgccaagcacctcctactttccaacaccatctggcagtatggtgacctctgatgcccagattttcaacaagccatactggctccaaagggctcaaggacacaacaatggcatctgttggagcaaccaactttttgtgacagtggtggacaccaccaggagcaccaatatgagtgtgtgttctgctgtgtcctcctctgacagcacctacaagaatgacaacttcaaggaatacctgagacatggagaggaatatgacctccaattcatcttccaactttgtaagattaccctgacagcagatgtgatgacctacatccacagtatgaacccaagcatcttggaggactggaactttggactgacacctcctccatctggcaccttggaggacacctacagatatgtgaccagccaggctgtgacttgtcagaagccatctgccccaaagccaaaggatgacccactgaaaaactacaccttctgggaggtggacctgaaagagaagttctctgctgacctggaccagtttccactgggcaggaagttcctgctccaagcaggactgaaagccagaccaaacttcagactgggcaagagggctgcccctgccagcaccagcaagaagtccagcaccaagaggaggaaggtgaagagctaaactcgagctc

SEQ ID NO: 74 - DNA, 1519 bp, Artificial sequence; identical to SEQ ID NO: 6
  3506 Synthetic HPV33 L1 gene

SEQ ID NO: 75 - DNA, 34 bp, Artificial sequence
  3507 HPV35L1 F1
cttggtaccatgagtctgtggaggagcaatgagg

SEQ ID NO: 76 - DNA, 36 bp, Artificial sequence; identical to SEQ ID NO: 34
  3508 HPV35L1 R1

SEQ ID NO: 77 - DNA, 1435 bp, Artificial sequence
  3509 HPV35L1 amplified sequence 1
cttggtaccatgagtctgtggaggagcaatgaggctacagtctacctgcctcctgtgtctgtgagcaaggtggtgagcacagatgaatatgtgaccaggaccaacatctactaccatgctggctccagcagactgctggctgtgggacacccatactatgccatcaagaagcaggacagcaacaagattgctgtgccaaaggtgtctggactccaatacagggtgttcagggtgaaactgcctgacccaaacaagtttggctttcctgacacctccttctatgaccctgccagccagagactggtgtgggcttgtactggagtggaggtgggcaggggacaaccactgggagtgggcatctctggacacccactgctgaacaaactggatgacacagagaacagcaacaaatatgtgggcaactctggcacagacaacagggagtgtatcagtatggactacaagcagacccaactttgtctgattggctgtagacctccaattggagaacactggggcaagggcacaccatgtaatgccaaccaggtgaaggctggagagtgtcctccattggaactgctgaacacagtgctccaagatggagatatggtggacacaggctttggagctatggacttcaccaccctccaagccaacaagtctgatgtgccactggacatctgttccagcatctgtaaataccctgactacctgaaaatggtgtctgaaccatatggagatatgctgttcttctacctgaggagggaacagatgtttgtgagacacctgttcaacagggctggcacagtgggagagacagtgcctgctgacctctacatcaagggcaccacaggcaccctgccaagcacctcctactttccaacaccatctggcagtatggtgacctctgatgcccagattttcaacaagccatactggctccaaagggctcaaggacacaacaatggcatctgttggagcaaccaactttttgtgacagtggtggacaccaccaggagcaccaatatgagtgtgtgttctgctgtgtcctcctctgacagcacctacaagaatgacaacttcaaggaatacctgagacatggagaggaatatgacctccaattcatcttccaactttgtaagattaccctgacagcagatgtgatgacctacatccacagtatgaacccaagcatcttggaggactggaactttggactgacacctcctccatctggcaccttggaggacacctacagatatgtgaccagccaggctgtgacttgtcagaagccatctgccccaaagccaaaggatgacccactgaaaaactacaccttctgggaggtggacctgaaagagaagttctctgctgacctggaccagtttccactgggcaggaagttcctgctccaagcaggactgaaagccaagc

SEQ ID NO: 78 - DNA, 35 bp, Artificial sequence; identical to SEQ ID NO: 36
  3510 HPV35L1 F2

SEQ ID NO: 79 - DNA, 36 bp, Artificial sequence; identical to SEQ ID NO: 37
  3511 HPV35L1 R2

SEQ ID NO: 80 - DNA, 101 bp, Artificial sequence; identical to SEQ ID NO: 38
  3512 HPV35L1 amplified sequence 2

SEQ ID NO: 81 - protein, 38 aa, Homo sapiens; identical to SEQ ID NO: 13
  3513 Amino acid sequence of HPV type 59 L1 protein aa 471-508

SEQ ID NO: 82 - protein, 469 aa, Homo sapiens
  3901 Amino acid sequence of HPV type 39 L1 protein aa 1-469
MAMWRSSDSMVYLPPPSVAKVVNTDDYVTRTGIYYYAGSSRLLTVGHPYFKVGMNGGRKQDIPKVSAYQYRVFRVTLPDPNKFSIPDASLYNPETQRLVWACVGVEVGRGQPLGVGISGHPLYNRQDDTENSPFSSTTNKDSRDNVSVDYKQTQLCIIGCVPAIGEHWGKGKACKPNNVSTGDCPPLELVNTPIEDGDMIDTGYGAMDFGALQETKSEVPLDICQSICKYPDYLQMSADVYGDSMFFCLRREQLFARHFWNRGGMVGDAIPAQLYIKGTDIRANPGSSVYCPSPSGSMVTSDSQLFNKPYWLHKAQGHNNGICWHNQLFLTVVDTTRSTNFTLSTSIESSIPSTYDPSKFKEYTRHVEEYDLQFIFQLCTVTLTTDVMSYIHTMNSSILDNWNFAVAPPPSASLVDTYRYLQSAAITCQKDAPAPEKKDPYDGLKFWNVDLREKFSLELDQFPLGRKFL

SEQ ID NO: 83 - protein, 38 aa, Homo sapiens; identical to SEQ ID NO: 13
  3902 Amino acid sequence of HPV type 59 L1 protein aa 471-508

SEQ ID NO: 84 - protein, 507 aa, Artificial sequence
  3903 Amino acid sequence of chimeric HPV type 39 L1 protein
MAMWRSSDSMVYLPPPSVAKVVNTDDYVTRTGIYYYAGSSRLLTVGHPYFKVGMNGGRKQDIPKVSAYQYRVFRVTLPDPNKFSIPDASLYNPETQRLVWACVGVEVGRGQPLGVGISGHPLYNRQDDTENSPFSSTTNKDSRDNVSVDYKQTQLCIIGCVPAIGEHWGKGKACKPNNVSTGDCPPLELVNTPIEDGDMIDTGYGAMDFGALQETKSEVPLDICQSICKYPDYLQMSADVYGDSMFFCLRREQLFARHFWNRGGMVGDAIPAQLYIKGTDIRANPGSSVYCPSPSGSMVTSDSQLFNKPYWLHKAQGHNNGICWHNQLFLTVVDTTRSTNFTLSTSIESSIPSTYDPSKFKEYTRHVEEYDLQFIFQLCTVTLTTDVMSYIHTMNSSILDNWNFAVAPPPSASLVDTYRYLQSAAITCQKDAPAPEKKDPYDGLKFWNVDLREKFSLELDQFPLGRKFLLQLGARPKPTIGPRKRAAPAPTSTPSPKRVKRRKSSRK

SEQ ID NO: 85 - DNA, 1525 bp, Artificial sequence
  3904 Nucleotide sequence of chimeric HPV type 39 L1 protein
atggctatgtggaggtcctctgacagtatggtctacctgcctcctccatctgtggctaaggtggtgaacacagatgactatgtgaccaggacaggcatctactactatgctggctccagcagactgctgacagtgggacacccatacttcaaggtggggatgaatggaggcaggaagcaggacatcccaaaggtgtctgcctaccaatacagggtgttcagggtgaccctgcctgacccaaacaagttcagcatccctgatgcctccctctacaaccctgagacccagagactggtgtgggcttgtgtgggagtggaggtgggcaggggacaaccactgggagtgggcatctctggacacccactctacaacagacaggatgacacagagaacagcccattctccagcaccaccaacaaggacagcagggacaatgtgtctgtggactacaagcagacccaactttgtatcattggctgtgtgcctgccattggagaacactggggcaagggcaaggcttgtaagccaaacaatgtgagcacaggagactgtcctccattggaactggtgaacacaccaattgaggatggagatatgattgacacaggctatggagctatggactttggagccctccaagagaccaagtctgaggtgccactggacatctgtcagagcatctgtaaataccctgactacctccaaatgagtgctgatgtctatggagacagtatgttcttctgtctgaggagggaacaactttttgccagacacttctggaacaggggagggatggtgggagatgccatccctgcccaactctacatcaagggcacagacatcagggctaaccctggctcctctgtctactgtccaagcccatctggcagtatggtgacctctgacagccaacttttcaacaagccatactggctgcacaaggctcaaggacacaacaatggcatctgttggcacaaccaacttttcctgacagtggtggacaccaccaggagcaccaacttcaccctgagcaccagcattgagtccagcatcccaagcacctatgacccaagcaagttcaaggaatacaccaggcatgtggaggaatatgacctccaattcatcttccaactttgtactgtgaccctgaccacagatgtgatgagttacatccacacaatgaactccagcatcctggacaactggaactttgctgtggctcctcctccatctgcctccctggtggacacctacagatacctccaatctgctgccatcacttgtcagaaggatgcccctgcccctgagaagaaggacccatatgatggactgaagttctggaatgtggacctgagggagaagttctccttggaactggaccagtttccactgggcaggaagttcctgctccaacttggagccagaccaaagccaaccattggaccaaggaagagggctgcccctgccccaaccagcacaccaagcccaaagagggtgaagaggaggaagtccagcaggaagtaaa

SEQ ID NO: 86 - DNA, 1537 bp, Artificial sequence
  3905 Synthetic HPV39 L1 gene
ctgggtaccatggctatgtggaggtcctctgacagtatggtctacctgcctcctccatctgtggctaaggtggtgaacacagatgactatgtgaccaggacaggcatctactactatgctggctccagcagactgctgacagtgggacacccatacttcaaggtggggatgaatggaggcaggaagcaggacatcccaaaggtgtctgcctaccaatacagggtgttcagggtgaccctgcctgacccaaacaagttcagcatccctgatgcctccctctacaaccctgagacccagagactggtgtgggcttgtgtgggagtggaggtgggcaggggacaaccactgggagtgggcatctctggacacccactctacaacagacaggatgacacagagaacagcccattctccagcaccaccaacaaggacagcagggacaatgtgtctgtggactacaagcagacccaactttgtatcattggctgtgtgcctgccattggagaacactggggcaagggcaaggcttgtaagccaaacaatgtgagcacaggagactgtcctccattggaactggtgaacacaccaattgaggatggagatatgattgacacaggctatggagctatggactttggagccctccaagagaccaagtctgaggtgccactggacatctgtcagagcatctgtaaataccctgactacctccaaatgagtgctgatgtctatggagacagtatgttcttctgtctgaggagggaacaactttttgccagacacttctggaacaggggagggatggtgggagatgccatccctgcccaactctacatcaagggcacagacatcagggctaaccctggctcctctgtctactgtccaagcccatctggcagtatggtgacctctgacagccaacttttcaacaagccatactggctgcacaaggctcaaggacacaacaatggcatctgttggcacaaccaacttttcctgacagtggtggacaccaccaggagcaccaacttcaccctgagcaccagcattgagtccagcatcccaagcacctatgacccaagcaagttcaaggaatacaccaggcatgtggaggaatatgacctccaattcatcttccaactttgtactgtgaccctgaccacagatgtgatgagttacatccacacaatgaactccagcatcctggacaactggaactttgctgtggctcctcctccatctgcctccctggtggacacctacagatacctccaatctgctgccatcacttgtcagaaggatgcccctgcccctgagaagaaggacccatatgatggactgaagttctggaatgtggacctgagggagaagttctccttggaactggaccagtttccactgggcaggaagttcctgctccaagccagggtgaggaggagaccaaccattggaccaaggaagagacctgctgccagcacctcctcctcctctgccaccaaacacaagaggaagagggtgagcaagtaaactcgagctc

SEQ ID NO: 87 - DNA, 1546 bp, Artificial sequence
  3906 Synthetic HPV59 L1 gene
ctgggtaccatggctctgtggaggtcctctgacaacaaggtctacctgcctcctccatctgtggctaaggtggtgagcacagatgaatatgtgaccaggaccagcatcttctaccatgctggctccagcagactgctgacagtgggacacccatacttcaaggtgccaaagggaggcaatggcagacaggatgtgccaaaggtgtctgcctaccaatacagggtgttcagggtgaaactgcctgacccaaacaagtttggactgcctgacaacacagtctatgacccaaacagccagagactggtgtgggcttgtgtgggagtggagattggcaggggacaaccactgggagtgggactgtctggacacccactctacaacaaactggatgacacagagaactctcatgtggcatctgctgtggacaccaaggacaccagggacaatgtgtctgtggactacaagcagacccaactttgtatcattggctgtgtgcctgccattggagaacactggaccaagggcacagcctgtaagccaaccacagtggtccagggagactgtcctccattggaactgataaacacaccaattgaggatggagatatggtggacacaggctatggagctatggacttcaaactgctccaagacaacaagtctgaggtgccactggacatctgtcagagcatctgtaaataccctgactacctccaaatgagtgctgatgcctatggagacagtatgttcttctgtctgaggagggaacaggtgtttgccagacacttctggaacaggtctggcacaatgggagaccaacttcctgagtccctctacatcaagggcacagacatcagggctaaccctggctcctacctctacagcccaagcccatctggctctgtggtgacctctgacagccaacttttcaacaagccatactggctgcacaaggctcaaggactgaacaatggcatctgttggcacaaccaacttttcctgacagtggtggacaccaccaggagcaccaacctgtctgtgtgtgccagcaccacctccagcatcccaaatgtctacacaccaacctccttcaaggaatatgccaggcatgtggaggagtttgacctccaattcatcttccaactttgtaagattaccctgaccacagaggtgatgagttacatccacaatatgaacaccaccatcttggaggactggaactttggagtgacacctcctccaacagcctccctggtggacacctacaggtttgtccagtctgctgctgtgacttgtcagaaggacacagcccctcctgtgaagcaggacccatatgacaaactgaagttctggcctgtggacctgaaagagaggttctctgctgacctggaccagtttccactgggcaggaagttcctgctccaacttggagccagaccaaagccaaccattggaccaaggaagagggctgcccctgccccaaccagcacaccaagcccaaagagggtgaagaggaggaagtccagcaggaagtaaactcgagctc

SEQ ID NO: 88 - DNA, 38 bp, Artificial sequence
  3907 HPV39L1 F1
cttggtaccatggctatgtggaggtcctctgacagtat

SEQ ID NO: 89 - DNA, 38 bp, Artificial sequence
  3908 HPV39L1 R1
tccaagttggagcaggaacttcctgcccagtggaaact

SEQ ID NO: 90 - DNA, 1428 bp, Artificial sequence
  3909 HPV39L1 amplified sequence 1
cttggtaccatggctatgtggaggtcctctgacagtatggtctacctgcctcctccatctgtggctaaggtggtgaacacagatgactatgtgaccaggacaggcatctactactatgctggctccagcagactgctgacagtgggacacccatacttcaaggtggggatgaatggaggcaggaagcaggacatcccaaaggtgtctgcctaccaatacagggtgttcagggtgaccctgcctgacccaaacaagttcagcatccctgatgcctccctctacaaccctgagacccagagactggtgtgggcttgtgtgggagtggaggtgggcaggggacaaccactgggagtgggcatctctggacacccactctacaacagacaggatgacacagagaacagcccattctccagcaccaccaacaaggacagcagggacaatgtgtctgtggactacaagcagacccaactttgtatcattggctgtgtgcctgccattggagaacactggggcaagggcaaggcttgtaagccaaacaatgtgagcacaggagactgtcctccattggaactggtgaacacaccaattgaggatggagatatgattgacacaggctatggagctatggactttggagccctccaagagaccaagtctgaggtgccactggacatctgtcagagcatctgtaaataccctgactacctccaaatgagtgctgatgtctatggagacagtatgttcttctgtctgaggagggaacaactttttgccagacacttctggaacaggggagggatggtgggagatgccatccctgcccaactctacatcaagggcacagacatcagggctaaccctggctcctctgtctactgtccaagcccatctggcagtatggtgacctctgacagccaacttttcaacaagccatactggctgcacaaggctcaaggacacaacaatggcatctgttggcacaaccaacttttcctgacagtggtggacaccaccaggagcaccaacttcaccctgagcaccagcattgagtccagcatcccaagcacctatgacccaagcaagttcaaggaatacaccaggcatgtggaggaatatgacctccaattcatcttccaactttgtactgtgaccctgaccacagatgtgatgagttacatccacacaatgaactccagcatcctggacaactggaactttgctgtggctcctcctccatctgcctccctggtggacacctacagatacctccaatctgctgccatcacttgtcagaaggatgcccctgcccctgagaagaaggacccatatgatggactgaagttctggaatgtggacctgagggagaagttctccttggaactggaccagtttccactgggcaggaagttcctgctccaacttgga

SEQ ID NO: 91 - DNA, 37 bp, Artificial sequence
  3910 HPV39L1 F2
aggaagttcctgctccaacttggagccagaccaaagc

SEQ ID NO: 92 - DNA, 40 bp, Artificial sequence
  3911 HPV39L1 R2
ctgtctagatttacttcctgctggacttcctcctcttcac

SEQ ID NO: 93 - DNA, 139 bp, Artificial sequence
  3912 HPV39L1 amplified sequence 2
aggaagttcctgctccaacttggagccagaccaaagccaaccattggaccaaggaagagggctgcccctgccccaaccagcacaccaagcccaaagagggtgaagaggaggaagtccagcaggaagtaaatctagacag

SEQ ID NO: 94 - protein, 26 aa, Homo sapiens
  3913 Amino acid sequence of HPV type 33 L1 protein aa 474-499
KAKPKLKRAAPTSTRTSSAKRKKVKK

SEQ ID NO: 95 - protein, 478 aa, Homo sapiens
  4501 Amino acid sequence of HPV type 45 L1 protein aa 1-478
MALWRPSDSTVYLPPPSVARVVNTDDYVSRTSIFYHAGSSRLLTVGNPYFRVVPSGAGNKQAVPKVSAYQYRVFRVALPDPNKFGLPDSTIYNPETQRLVWACVGMEIGRGQPLGIGLSGHPFYNKLDDTESAHAATAVITQDVRDNVSVDYKQTQLCILGCVPAIGEHWAKGTLCKPAQLQPGDCPPLELKNTIIEDGDMVDTGYGAMDFSTLQDTKCEVPLDICQSICKYPDYLQMSADPYGDSMFFCLRREQLFARHFWNRAGVMGDTVPTDLYIKGTSANMRETPGSCVYSPSPSGSITTSDSQLFNKPYWLHKAQGHNNGICWHNQLFVTVVDTTRSTNLTLCASTQNPVPNTYDPTKFKHYSRHVEEYDLQFIFQLCTITLTAEVMSYIHSMNSSILENWNFGVPPPPTTSLVDTYRFVQSVAVTCQKDTTPPEKQDPYDKLKFWTVDLKEKFSSDLDQYPLGRKFLVQAGL

SEQ ID NO: 96 - protein, 26 aa, Homo sapiens
  4502 Amino acid sequence of HPV type 33 L1 protein aa 474-499
KAKPKLKRAAPTSTRTSSAKRKKVKK

SEQ ID NO: 97 - protein, 504 aa, Artificial sequence
  4503 Amino acid sequence of chimeric HPV type 45 L1 protein
MALWRPSDSTVYLPPPSVARVVNTDDYVSRTSIFYHAGSSRLLTVGNPYFRVVPSGAGNKQAVPKVSAYQYRVFRVALPDPNKFGLPDSTIYNPETQRLVWACVGMEIGRGQPLGIGLSGHPFYNKLDDTESAHAATAVITQDVRDNVSVDYKQTQLCILGCVPAIGEHWAKGTLCKPAQLQPGDCPPLELKNTIIEDGDMVDTGYGAMDFSTLQDTKCEVPLDICQSICKYPDYLQMSADPYGDSMFFCLRREQLFARHFWNRAGVMGDTVPTDLYIKGTSANMRETPGSCVYSPSPSGSITTSDSQLFNKPYWLHKAQGHNNGICWHNQLFVTVVDTTRSTNLTLCASTQNPVPNTYDPTKFKHYSRHVEEYDLQFIFQLCTITLTAEVMSYIHSMNSSILENWNFGVPPPPTTSLVDTYRFVQSVAVTCQKDTTPPEKQDPYDKLKFWTVDLKEKFSSDLDQYPLGRKFLVQAGLKAKPKLKRAAPTSTRTSSAKRKKVKK

SEQ ID NO: 98 - DNA, 1516 bp, Artificial sequence
  4504 Nucleotide sequence of chimeric HPV type 45 L1 protein
atggctctgtggagaccatctgacagcacagtctacctgcctcctccatctgtggcaagggtggtgaacacagatgactatgtgagcaggaccagcatcttctaccatgctggctccagcagactgctgacagtgggcaacccatacttcagggtggtgccaagtggagcaggcaacaagcaggctgtgccaaaggtgtctgcctaccaatacagggtgttcagggtggctctgcctgacccaaacaagtttggactgcctgacagcaccatctacaaccctgagacccagagactggtgtgggcttgtgtggggatggagattggcaggggacaaccactgggcattggactgtctggacacccattctacaacaaactggatgacacagagtctgcccatgctgccacagcagtgattacccaggatgtgagggacaatgtgtctgtggactacaagcagacccaactttgtatcctgggctgtgtgcctgccattggagaacactgggctaagggcaccctgtgtaagcctgcccaactccaacctggagactgtcctccattggaactgaaaaacaccatcattgaggatggagatatggtggacacaggctatggagctatggacttcagcaccctccaagacaccaagtgtgaggtgccactggacatctgtcagagcatctgtaaataccctgactacctccaaatgagtgctgacccatatggagacagtatgttcttctgtctgaggagggaacaactttttgccagacacttctggaacagggctggagtgatgggagacacagtgccaacagacctctacatcaagggcacctctgccaatatgagggagacacctggctcctgtgtctacagcccaagcccatctggcagcatcaccacctctgacagccaacttttcaacaagccatactggctgcacaaggctcaaggacacaacaatggcatctgttggcacaaccaactttttgtgacagtggtggacaccaccaggagcaccaacctgaccctgtgtgccagcacccagaaccctgtgccaaacacctatgacccaaccaagttcaagcactacagcaggcatgtggaggaatatgacctccaattcatcttccaactttgtaccatcaccctgacagcagaggtgatgagttacatccacagtatgaactccagcatcttggagaactggaactttggagtgcctcctcctccaaccacctccctggtggacacctacaggtttgtccagtctgtggctgtgacttgtcagaaggacaccacacctcctgagaagcaggacccatatgacaaactgaagttctggacagtggacctgaaagagaagttctcctctgacctggaccaatacccactgggcaggaagttcctggtccaggctggactgaaagccaagccaaaactgaaaagggctgccccaaccagcaccaggacctcctctgccaagaggaagaaggtgaagaagtaaa

SEQ ID NO: 99 - DNA, 1552 bp, Artificial sequence
  4505 Synthetic HPV45 L1 gene
ctgggtaccatggctctgtggagaccatctgacagcacagtctacctgcctcctccatctgtggcaagggtggtgaacacagatgactatgtgagcaggaccagcatcttctaccatgctggctccagcagactgctgacagtgggcaacccatacttcagggtggtgccaagtggagcaggcaacaagcaggctgtgccaaaggtgtctgcctaccaatacagggtgttcagggtggctctgcctgacccaaacaagtttggactgcctgacagcaccatctacaaccctgagacccagagactggtgtgggcttgtgtggggatggagattggcaggggacaaccactgggcattggactgtctggacacccattctacaacaaactggatgacacagagtctgcccatgctgccacagcagtgattacccaggatgtgagggacaatgtgtctgtggactacaagcagacccaactttgtatcctgggctgtgtgcctgccattggagaacactgggctaagggcaccctgtgtaagcctgcccaactccaacctggagactgtcctccattggaactgaaaaacaccatcattgaggatggagatatggtggacacaggctatggagctatggacttcagcaccctccaagacaccaagtgtgaggtgccactggacatctgtcagagcatctgtaaataccctgactacctccaaatgagtgctgacccatatggagacagtatgttcttctgtctgaggagggaacaactttttgccagacacttctggaacagggctggagtgatgggagacacagtgccaacagacctctacatcaagggcacctctgccaatatgagggagacacctggctcctgtgtctacagcccaagcccatctggcagcatcaccacctctgacagccaacttttcaacaagccatactggctgcacaaggctcaaggacacaacaatggcatctgttggcacaaccaactttttgtgacagtggtggacaccaccaggagcaccaacctgaccctgtgtgccagcacccagaaccctgtgccaaacacctatgacccaaccaagttcaagcactacagcaggcatgtggaggaatatgacctccaattcatcttccaactttgtaccatcaccctgacagcagaggtgatgagttacatccacagtatgaactccagcatcttggagaactggaactttggagtgcctcctcctccaaccacctccctggtggacacctacaggtttgtccagtctgtggctgtgacttgtcagaaggacaccacacctcctgagaagcaggacccatatgacaaactgaagttctggacagtggacctgaaagagaagttctcctctgacctggaccaatacccactgggcaggaagttcctggtccaggctggactgaggaggagaccaaccattggaccaaggaagagacctgctgccagcaccagcacagccagcagacctgccaagagggtgaggattaggagcaagaagtaaactcgagctc

SEQ ID NO: 100 - DNA, 1519 bp, Artificial sequence; identical to SEQ ID NO: 6
  4506 Synthetic HPV33 L1 gene

SEQ ID NO: 101 - DNA, 33 bp, Artificial sequence
  4507 HPV45L1 F1
cttggtaccatggctctgtggagaccatctgac

SEQ ID NO: 102 - DNA, 32 bp, Artificial sequence
  4508 HPV45L1 R1
gcttggctttcagtccagcctggaccaggaac

SEQ ID NO: 103 - DNA, 1453 bp, Artificial sequence
  4509 HPV45L1 amplified sequence 1
cttggtaccatggctctgtggagaccatctgacagcacagtctacctgcctcctccatctgtggcaagggtggtgaacacagatgactatgtgagcaggaccagcatcttctaccatgctggctccagcagactgctgacagtgggcaacccatacttcagggtggtgccaagtggagcaggcaacaagcaggctgtgccaaaggtgtctgcctaccaatacagggtgttcagggtggctctgcctgacccaaacaagtttggactgcctgacagcaccatctacaaccctgagacccagagactggtgtgggcttgtgtggggatggagattggcaggggacaaccactgggcattggactgtctggacacccattctacaacaaactggatgacacagagtctgcccatgctgccacagcagtgattacccaggatgtgagggacaatgtgtctgtggactacaagcagacccaactttgtatcctgggctgtgtgcctgccattggagaacactgggctaagggcaccctgtgtaagcctgcccaactccaacctggagactgtcctccattggaactgaaaaacaccatcattgaggatggagatatggtggacacaggctatggagctatggacttcagcaccctccaagacaccaagtgtgaggtgccactggacatctgtcagagcatctgtaaataccctgactacctccaaatgagtgctgacccatatggagacagtatgttcttctgtctgaggagggaacaactttttgccagacacttctggaacagggctggagtgatgggagacacagtgccaacagacctctacatcaagggcacctctgccaatatgagggagacacctggctcctgtgtctacagcccaagcccatctggcagcatcaccacctctgacagccaacttttcaacaagccatactggctgcacaaggctcaaggacacaacaatggcatctgttggcacaaccaactttttgtgacagtggtggacaccaccaggagcaccaacctgaccctgtgtgccagcacccagaaccctgtgccaaacacctatgacccaaccaagttcaagcactacagcaggcatgtggaggaatatgacctccaattcatcttccaactttgtaccatcaccctgacagcagaggtgatgagttacatccacagtatgaactccagcatcttggagaactggaactttggagtgcctcctcctccaaccacctccctggtggacacctacaggtttgtccagtctgtggctgtgacttgtcagaaggacaccacacctcctgagaagcaggacccatatgacaaactgaagttctggacagtggacctgaaagagaagttctcctctgacctggaccaatacccactgggcaggaagttcctggtccaggctggactgaaagccaagc

SEQ ID NO: 104 - DNA, 35 bp, Artificial sequence
  4510 HPV45L1 F2
ggctggactgaaagccaagccaaaactgaaaaggg

SEQ ID NO: 105 - DNA, 37 bp, Artificial sequence; identical to SEQ ID NO: 11
  4511 HPV45L1 R2

SEQ ID NO: 106 - DNA, 101 bp, Artificial sequence
  4512 HPV45L1 amplified sequence 2
ggctggactgaaagccaagccaaaactgaaaagggctgccccaaccagcaccaggacctcctctgccaagaggaagaaggtgaagaagtaaatctagacag

SEQ ID NO: 107 - protein, 38 aa, Homo sapiens; identical to SEQ ID NO: 13
  4513 Amino acid sequence of HPV type 59 L1 protein aa 471-508

SEQ ID NO: 108 - protein, 474 aa, Homo sapiens
  5101 Amino acid sequence of HPV type 51 L1 protein aa 1-474
MALWRTNDSKVYLPPAPVSRIVNTEEYITRTGIYYYAGSSRLITLGHPYFPIPKTSTRAAIPKVSAFQYRVFRVQLPDPNKFGLPDPNLYNPDTDRLVWGCVGVEVGRGQPLGVGLSGHPLFNKYDDTENSRIANGNAQQDVRDNTSVDNKQTQLCIIGCAPPIGEHWGIGTTCKNTPVPPGDCPPLELVSSVIQDGDMIDTGFGAMDFAALQATKSDVPLDISQSVCKYPDYLKMSADTYGNSMFFHLRREQIFARHYYNKLVGVGEDIPNDYYIKGSGNGRDPIESYIYSATPSGSMITSDSQIFNKPYWLHRAQGHNNGICWNNQLFITCVDTTRSTNLTISTATAAVSPTFTPSNFKQYIRHGEEYELQFIFQLCKITLTTEVMAYLHTMDPTILEQWNFGLTLPPSASLEDAYRFVRNAATSCQKDTPPQAKPDPLAKYKFWDVDLKERFSLDLDQFALGRKFLLQVGV

SEQ ID NO: 109 - protein, 26 aa, Homo sapiens
  5102 Amino acid sequence of HPV type 33 L1 protein aa 474-499
KAKPKLKRAAPTSTRTSSAKRKKVKK

SEQ ID NO: 110 - protein, 500 aa, Artificial sequence
  5103 Amino acid sequence of chimeric HPV type 51 L1 protein
MALWRTNDSKVYLPPAPVSRIVNTEEYITRTGIYYYAGSSRLITLGHPYFPIPKTSTRAAIPKVSAFQYRVFRVQLPDPNKFGLPDPNLYNPDTDRLVWGCVGVEVGRGQPLGVGLSGHPLFNKYDDTENSRIANGNAQQDVRDNTSVDNKQTQLCIIGCAPPIGEHWGIGTTCKNTPVPPGDCPPLELVSSVIQDGDMIDTGFGAMDFAALQATKSDVPLDISQSVCKYPDYLKMSADTYGNSMFFHLRREQIFARHYYNKLVGVGEDIPNDYYIKGSGNGRDPIESYIYSATPSGSMITSDSQIFNKPYWLHRAQGHNNGICWNNQLFITCVDTTRSTNLTISTATAAVSPTFTPSNFKQYIRHGEEYELQFIFQLCKITLTTEVMAYLHTMDPTILEQWNFGLTLPPSASLEDAYRFVRNAATSCQKDTPPQAKPDPLAKYKFWDVDLKERFSLDLDQFALGRKFLLQVGVKAKPKLKRAAPTSTRTSSAKRKKVKK

SEQ ID NO: 111 - DNA, 1504 bp, Artificial sequence
  5104 Nucleotide sequence of chimeric HPV type 51 L1 protein
atggctctgtggaggaccaatgacagcaaggtctacctgcctcctgcccctgtgagcaggattgtgaacacagaggaatacatcaccaggacaggcatctactactatgctggctccagcagactgattaccctgggacacccatactttccaatcccaaagaccagcaccagggctgccatcccaaaggtgtctgccttccaatacagggtgttcagggtccaacttcctgacccaaacaagtttggactgcctgacccaaacctctacaaccctgacacagacagactggtgtggggctgtgtgggagtggaggtgggcaggggacaaccactgggagtgggactgtctggacacccactgttcaacaaatatgatgacacagagaacagcaggattgccaatggcaatgcccaacaggatgtgagggacaacacctctgtggacaacaagcagacccaactttgtatcattggctgtgcccctccaattggagaacactggggcattggcaccacttgtaagaacacacctgtgcctcctggagactgtcctccattggaactggtgtcctctgtgattcaggatggagatatgattgacacaggctttggagctatggactttgctgccctccaagccaccaagtctgatgtgccactggacatcagccagtctgtgtgtaaataccctgactacctgaaaatgagtgctgacacctatggcaacagtatgttcttccacctgaggagggaacagatttttgccagacactactacaacaaactggtgggagtgggagaggacatcccaaatgactactacatcaagggctctggcaatggcagggacccaattgagtcctacatctactctgccacaccatctggcagtatgattacctctgacagccagattttcaacaagccatactggctgcacagggctcaaggacacaacaatggcatctgttggaacaaccaacttttcatcacttgtgtggacaccaccaggagcaccaacctgaccatcagcacagccacagcagcagtgagcccaaccttcacaccaagcaacttcaagcaatacatcagacatggagaggaatatgaactccaattcatcttccaactttgtaagattaccctgaccacagaggtgatggcttacctgcacacaatggacccaaccatcttggaacagtggaactttggactgaccctgcctccatctgcctccttggaggatgcctacaggtttgtgaggaatgctgccacctcctgtcagaaggacacacctccacaggctaagcctgacccactggctaaatacaagttctgggatgtggacctgaaagagaggttctccctggacctggaccagtttgccctgggcaggaagttcctgctccaagtgggagtcaaagccaagccaaaactgaaaagggctgccccaaccagcaccaggacctcctctgccaagaggaagaaggtgaagaagtaaa

SEQ ID NO: 112 - DNA, 1534 bp, Artificial sequence
  5105 Synthetic HPV51 L1 gene
ctgggtaccatggctctgtggaggaccaatgacagcaaggtctacctgcctcctgcccctgtgagcaggattgtgaacacagaggaatacatcaccaggacaggcatctactactatgctggctccagcagactgattaccctgggacacccatactttccaatcccaaagaccagcaccagggctgccatcccaaaggtgtctgccttccaatacagggtgttcagggtccaacttcctgacccaaacaagtttggactgcctgacccaaacctctacaaccctgacacagacagactggtgtggggctgtgtgggagtggaggtgggcaggggacaaccactgggagtgggactgtctggacacccactgttcaacaaatatgatgacacagagaacagcaggattgccaatggcaatgcccaacaggatgtgagggacaacacctctgtggacaacaagcagacccaactttgtatcattggctgtgcccctccaattggagaacactggggcattggcaccacttgtaagaacacacctgtgcctcctggagactgtcctccattggaactggtgtcctctgtgattcaggatggagatatgattgacacaggctttggagctatggactttgctgccctccaagccaccaagtctgatgtgccactggacatcagccagtctgtgtgtaaataccctgactacctgaaaatgagtgctgacacctatggcaacagtatgttcttccacctgaggagggaacagatttttgccagacactactacaacaaactggtgggagtgggagaggacatcccaaatgactactacatcaagggctctggcaatggcagggacccaattgagtcctacatctactctgccacaccatctggcagtatgattacctctgacagccagattttcaacaagccatactggctgcacagggctcaaggacacaacaatggcatctgttggaacaaccaacttttcatcacttgtgtggacaccaccaggagcaccaacctgaccatcagcacagccacagcagcagtgagcccaaccttcacaccaagcaacttcaagcaatacatcagacatggagaggaatatgaactccaattcatcttccaactttgtaagattaccctgaccacagaggtgatggcttacctgcacacaatggacccaaccatcttggaacagtggaactttggactgaccctgcctccatctgcctccttggaggatgcctacaggtttgtgaggaatgctgccacctcctgtcagaaggacacacctccacaggctaagcctgacccactggctaaatacaagttctgggatgtggacctgaaagagaggttctccctggacctggaccagtttgccctgggcaggaagttcctgctccaagtgggagtccagaggaagccaagacctggactgaaaagacctgcctcctctgcctcctcctcctcctcctcctctgccaagaggaagagggtgaagaagtaaactcgagctc

SEQ ID NO: 113 - DNA, 1519 bp, Artificial sequence; identical to SEQ ID NO: 6
  5106 Synthetic HPV33 L1 gene

SEQ ID NO: 114 - DNA, 34 bp, Artificial sequence
  5107 HPV51L1 F1
cttggtaccatggctctgtggaggaccaatgaca

SEQ ID NO: 115 - DNA, 32 bp, Artificial sequence
  5108 HPV51L1 R1
gcttggctttgactcccacttggagcaggaac

SEQ ID NO: 116 - DNA, 1441 bp, Artificial sequence
  5109 HPV51L1 amplified sequence 1
cttggtaccatggctctgtggaggaccaatgacagcaaggtctacctgcctcctgcccctgtgagcaggattgtgaacacagaggaatacatcaccaggacaggcatctactactatgctggctccagcagactgattaccctgggacacccatactttccaatcccaaagaccagcaccagggctgccatcccaaaggtgtctgccttccaatacagggtgttcagggtccaacttcctgacccaaacaagtttggactgcctgacccaaacctctacaaccctgacacagacagactggtgtggggctgtgtgggagtggaggtgggcaggggacaaccactgggagtgggactgtctggacacccactgttcaacaaatatgatgacacagagaacagcaggattgccaatggcaatgcccaacaggatgtgagggacaacacctctgtggacaacaagcagacccaactttgtatcattggctgtgcccctccaattggagaacactggggcattggcaccacttgtaagaacacacctgtgcctcctggagactgtcctccattggaactggtgtcctctgtgattcaggatggagatatgattgacacaggctttggagctatggactttgctgccctccaagccaccaagtctgatgtgccactggacatcagccagtctgtgtgtaaataccctgactacctgaaaatgagtgctgacacctatggcaacagtatgttcttccacctgaggagggaacagatttttgccagacactactacaacaaactggtgggagtgggagaggacatcccaaatgactactacatcaagggctctggcaatggcagggacccaattgagtcctacatctactctgccacaccatctggcagtatgattacctctgacagccagattttcaacaagccatactggctgcacagggctcaaggacacaacaatggcatctgttggaacaaccaacttttcatcacttgtgtggacaccaccaggagcaccaacctgaccatcagcacagccacagcagcagtgagcccaaccttcacaccaagcaacttcaagcaatacatcagacatggagaggaatatgaactccaattcatcttccaactttgtaagattaccctgaccacagaggtgatggcttacctgcacacaatggacccaaccatcttggaacagtggaactttggactgaccctgcctccatctgcctccttggaggatgcctacaggtttgtgaggaatgctgccacctcctgtcagaaggacacacctccacaggctaagcctgacccactggctaaatacaagttctgggatgtggacctgaaagagaggttctccctggacctggaccagtttgccctgggcaggaagttcctgctccaagtgggagtcaaagccaagc

SEQ ID NO: 117 - DNA, 35 bp, Artificial sequence
  5110 HPV51L1 F2
agtgggagtcaaagccaagccaaaactgaaaaggg

SEQ ID NO: 118 - DNA, 36 bp, Artificial sequence; identical to SEQ ID NO: 37
  5111 HPV51L1 R2

SEQ ID NO: 119 - DNA, 101 bp, Artificial sequence
  5112 HPV51L1 amplified sequence 2
agtgggagtcaaagccaagccaaaactgaaaagggctgccccaaccagcaccaggacctcctctgccaagaggaagaaggtgaagaagtaaatctagacag

SEQ ID NO: 120 - protein, 38 aa, Homo sapiens; identical to SEQ ID NO: 13
  5113 Amino acid sequence of HPV type 59 L1 protein aa 471-508

SEQ ID NO: 121 - protein, 478 aa, Homo sapiens
  5201 Amino acid sequence of HPV type 52 L1 protein aa 1-478
MSVWRPSEATVYLPPVPVSKVVSTDEYVSRTSIYYYAGSSRLLTVGHPYFSIKNTSSGNGKKVLVPKVSGLQYRVFRIKLPDPNKFGFPDTSFYNPETQRLVWACTGLEIGRGQPLGVGISGHPLLNKFDDTETSNKYAGKPGIDNRECLSMDYKQTQLCILGCKPPIGEHWGKGTPCNNNSGNPGDCPPLQLINSVIQDGDMVDTGFGCMDFNTLQASKSDVPIDICSSVCKYPDYLQMASEPYGDSLFFFLRREQMFVRHFFNRAGTLGDPVPGDLYIQGSNSGNTATVQSSAFFPTPSGSMVTSESQLFNKPYWLQRAQGHNNGICWGNQLFVTVVDTTRSTNMTLCAEVKKESTYKNENFKEYLRHGEEFDLQFIFQLCKITLTADVMTYIHKMDATILEDWQFGLTPPPSASLEDTYRFVTSTAITCQKNTPPKGKEDPLKDYMFWEVDLKEKFSADLDQFPLGRKFLLQAGL

SEQ ID NO: 122 - protein, 26 aa, Homo sapiens
  5202 Amino acid sequence of HPV type 33 L1 protein aa 474-499
KAKPKLKRAAPTSTRTSSAKRKKVKK

SEQ ID NO: 123 - protein, 504 aa, Artificial sequence
  5203 Amino acid sequence of chimeric HPV type 52 L1 protein
MSVWRPSEATVYLPPVPVSKVVSTDEYVSRTSIYYYAGSSRLLTVGHPYFSIKNTSSGNGKKVLVPKVSGLQYRVFRIKLPDPNKFGFPDTSFYNPETQRLVWACTGLEIGRGQPLGVGISGHPLLNKFDDTETSNKYAGKPGIDNRECLSMDYKQTQLCILGCKPPIGEHWGKGTPCNNNSGNPGDCPPLQLINSVIQDGDMVDTGFGCMDFNTLQASKSDVPIDICSSVCKYPDYLQMASEPYGDSLFFFLRREQMFVRHFFNRAGTLGDPVPGDLYIQGSNSGNTATVQSSAFFPTPSGSMVTSESQLFNKPYWLQRAQGHNNGICWGNQLFVTVVDTTRSTNMTLCAEVKKESTYKNENFKEYLRHGEEFDLQFIFQLCKITLTADVMTYIHKMDATILEDWQFGLTPPPSASLEDTYRFVTSTAITCQKNTPPKGKEDPLKDYMFWEVDLKEKFSADLDQFPLGRKFLLQAGLKAKPKLKRAAPTSTRTSSAKRKKVKK

SEQ ID NO: 124 - DNA, 1516 bp, Artificial sequence
  5204 Nucleotide sequence of chimeric HPV type 52 L1 protein
atgagcgtgtggaggcccagcgaggccaccgtgtacctgccccccgtgcccgtgagcaaggtggtgagcaccgacgagtacgtgagcaggaccagcatctactactacgccggcagcagcaggctgctgaccgtgggccacccctacttcagcatcaagaacaccagcagcggcaacggcaagaaggtgctggtgcccaaggtgagcggcctgcagtacagggtgttcaggatcaagctgcccgaccccaacaagttcggcttccccgacaccagcttctacaaccccgagacccagaggctggtgtgggcctgcaccggcctggagatcggcaggggccagcccctgggcgtgggcatcagcggccaccccctgctgaacaagttcgacgacaccgagaccagcaacaagtacgccggcaagcccggcatcgacaacagggagtgcctgagcatggactacaagcagacccagctgtgcatcctgggctgcaagccccccatcggcgagcactggggcaagggcaccccctgcaacaacaacagcggcaaccccggcgactgcccccccctgcagctgatcaacagcgtgatccaggacggcgacatggtggacaccggcttcggctgcatggacttcaacaccctgcaggccagcaagagcgacgtgcccatcgacatctgcagcagcgtgtgcaagtaccccgactacctgcagatggccagcgagccctacggcgacagcctgttcttcttcctgaggagggagcagatgttcgtgaggcacttcttcaacagggccggcaccctgggcgaccccgtgcccggcgacctgtacatccagggcagcaacagcggcaacaccgccaccgtgcagagcagcgccttcttccccacccccagcggcagcatggtgaccagcgagagccagctgttcaacaagccctactggctgcagagggcccagggccacaacaacggcatctgctggggcaaccagctgttcgtgaccgtggtggacaccaccaggagcaccaacatgaccctgtgcgccgaggtgaagaaggagagcacctacaagaacgagaacttcaaggagtacctgaggcacggcgaggagttcgacctgcagttcatcttccagctgtgcaagatcaccctgaccgccgacgtgatgacctacatccacaagatggacgccaccatcctggaggactggcagttcggcctgacccccccccccagcgccagcctggaggacacctacaggttcgtgaccagcaccgccatcacctgccagaagaacaccccccccaagggcaaggaggaccccctgaaggactacatgttctgggaggtggacctgaaggagaagttcagcgccgacctggaccagttccccctgggcaggaagttcctgctgcaggccggcctgaaagccaagccaaaactgaaaagggctgccccaaccagcaccaggacctcctctgccaagaggaagaaggtgaagaagtaaa

SEQ ID NO: 125 - DNA, 1531 bp, Artificial sequence
  5205 Synthetic HPV52 L1 gene
ctgggtaccatgagcgtgtggaggcccagcgaggccaccgtgtacctgccccccgtgcccgtgagcaaggtggtgagcaccgacgagtacgtgagcaggaccagcatctactactacgccggcagcagcaggctgctgaccgtgggccacccctacttcagcatcaagaacaccagcagcggcaacggcaagaaggtgctggtgcccaaggtgagcggcctgcagtacagggtgttcaggatcaagctgcccgaccccaacaagttcggcttccccgacaccagcttctacaaccccgagacccagaggctggtgtgggcctgcaccggcctggagatcggcaggggccagcccctgggcgtgggcatcagcggccaccccctgctgaacaagttcgacgacaccgagaccagcaacaagtacgccggcaagcccggcatcgacaacagggagtgcctgagcatggactacaagcagacccagctgtgcatcctgggctgcaagccccccatcggcgagcactggggcaagggcaccccctgcaacaacaacagcggcaaccccggcgactgcccccccctgcagctgatcaacagcgtgatccaggacggcgacatggtggacaccggcttcggctgcatggacttcaacaccctgcaggccagcaagagcgacgtgcccatcgacatctgcagcagcgtgtgcaagtaccccgactacctgcagatggccagcgagccctacggcgacagcctgttcttcttcctgaggagggagcagatgttcgtgaggcacttcttcaacagggccggcaccctgggcgaccccgtgcccggcgacctgtacatccagggcagcaacagcggcaacaccgccaccgtgcagagcagcgccttcttccccacccccagcggcagcatggtgaccagcgagagccagctgttcaacaagccctactggctgcagagggcccagggccacaacaacggcatctgctggggcaaccagctgttcgtgaccgtggtggacaccaccaggagcaccaacatgaccctgtgcgccgaggtgaagaaggagagcacctacaagaacgagaacttcaaggagtacctgaggcacggcgaggagttcgacctgcagttcatcttccagctgtgcaagatcaccctgaccgccgacgtgatgacctacatccacaagatggacgccaccatcctggaggactggcagttcggcctgacccccccccccagcgccagcctggaggacacctacaggttcgtgaccagcaccgccatcacctgccagaagaacaccccccccaagggcaaggaggaccccctgaaggactacatgttctgggaggtggacctgaaggagaagttcagcgccgacctggaccagttccccctgggcaggaagttcctgctgcaggccggcctgcaggccaggcccaagctgaagaggcccgccagcagcgcccccaggaccagcaccaagaagaagaaggtgaagaggtaaactcgagctc

SEQ ID NO: 126 - DNA, 1519 bp, Artificial sequence; identical to SEQ ID NO: 6
  5206 Synthetic HPV33 L1 gene

SEQ ID NO: 127 - DNA, 34 bp, Artificial sequence
  5207 HPV52L1 F1
cttggtaccatgagcgtgtggaggcccagcgagg

SEQ ID NO: 128 - DNA, 35 bp, Artificial sequence
  5208 HPV52L1 R1
gcttggctttcaggccggcctgcagcaggaacttc

SEQ ID NO: 129 - DNA, 1453 bp, Artificial sequence
  5209 HPV52L1 amplified sequence 1
cttggtaccatgagcgtgtggaggcccagcgaggccaccgtgtacctgccccccgtgcccgtgagcaaggtggtgagcaccgacgagtacgtgagcaggaccagcatctactactacgccggcagcagcaggctgctgaccgtgggccacccctacttcagcatcaagaacaccagcagcggcaacggcaagaaggtgctggtgcccaaggtgagcggcctgcagtacagggtgttcaggatcaagctgcccgaccccaacaagttcggcttccccgacaccagcttctacaaccccgagacccagaggctggtgtgggcctgcaccggcctggagatcggcaggggccagcccctgggcgtgggcatcagcggccaccccctgctgaacaagttcgacgacaccgagaccagcaacaagtacgccggcaagcccggcatcgacaacagggagtgcctgagcatggactacaagcagacccagctgtgcatcctgggctgcaagccccccatcggcgagcactggggcaagggcaccccctgcaacaacaacagcggcaaccccggcgactgcccccccctgcagctgatcaacagcgtgatccaggacggcgacatggtggacaccggcttcggctgcatggacttcaacaccctgcaggccagcaagagcgacgtgcccatcgacatctgcagcagcgtgtgcaagtaccccgactacctgcagatggccagcgagccctacggcgacagcctgttcttcttcctgaggagggagcagatgttcgtgaggcacttcttcaacagggccggcaccctgggcgaccccgtgcccggcgacctgtacatccagggcagcaacagcggcaacaccgccaccgtgcagagcagcgccttcttccccacccccagcggcagcatggtgaccagcgagagccagctgttcaacaagccctactggctgcagagggcccagggccacaacaacggcatctgctggggcaaccagctgttcgtgaccgtggtggacaccaccaggagcaccaacatgaccctgtgcgccgaggtgaagaaggagagcacctacaagaacgagaacttcaaggagtacctgaggcacggcgaggagttcgacctgcagttcatcttccagctgtgcaagatcaccctgaccgccgacgtgatgacctacatccacaagatggacgccaccatcctggaggactggcagttcggcctgacccccccccccagcgccagcctggaggacacctacaggttcgtgaccagcaccgccatcacctgccagaagaacaccccccccaagggcaaggaggaccccctgaaggactacatgttctgggaggtggacctgaaggagaagttcagcgccgacctggaccagttccccctgggcaggaagttcctgctgcaggccggcctgaaagccaagc

SEQ ID NO: 130 - DNA, 35 bp, Artificial sequence
  5210 HPV52L1 F2
ggccggcctgaaagccaagccaaaactgaaaaggg

SEQ ID NO: 131 - DNA, 36 bp, Artificial sequence; identical to SEQ ID NO: 37
  5211 HPV52L1 R2

SEQ ID NO: 132 - DNA, 101 bp, Artificial sequence
  5212 HPV52L1 amplified sequence 2
ggccggcctgaaagccaagccaaaactgaaaagggctgccccaaccagcaccaggacctcctctgccaagaggaagaaggtgaagaagtaaatctagacag

SEQ ID NO: 133 - protein, 38 aa, Homo sapiens; identical to SEQ ID NO: 13
  5213 Amino acid sequence of HPV type 59 L1 protein aa 471-508

SEQ ID NO: 134 - protein, 467 aa, Homo sapiens
  5601 Amino acid sequence of HPV type 56 L1 protein aa 1-467
MATWRPSENKVYLPPTPVSKVVATDSYVKRTSIFYHAGSSRLLAVGHPYYSVTKDNTKTNIPKVSAYQYRVFRVRLPDPNKFGLPDTNIYNPDQERLVWACVGLEVGRGQPLGAGLSGHPLFNRLDDTESSNLANNNVIEDSRDNISVDGKQTQLCIVGCTPAMGEHWTKGAVCKSTQVTTGDCPPLALINTPIEDGDMIDTGFGAMDFKVLQESKAEVPLDIVQSTCKYPDYLKMSADAYGDSMWFYLRREQLFARHYFNRAGKVGETIPAELYLKGSNGREPPPSSVYVATPSGSMITSEAQLFNKPYWLQRAQGHNNGICWGNQLFVTVVDTTRSTNMTISTATEQLSKYDARKINQYLRHVEEYELQFVFQLCKITLSAEVMAYLHNMNANLLEDWNIGLSPPVATSLEDKYRYVRSTAITCQREQPPTEKQDPLAKYKFWDVNLQDSFSTDLDQFPLGRKFL

SEQ ID NO: 135 - protein, 31 aa, Homo sapiens
  5602 Amino acid sequence of HPV type 33 L1 protein aa 469-499
LQAGLKAKPKLKRAAPTSTRTSSAKRKKVKK

SEQ ID NO: 136 - protein, 498 aa, Artificial sequence
  5603 Amino acid sequence of chimeric HPV type 56 L1 protein
MATWRPSENKVYLPPTPVSKVVATDSYVKRTSIFYHAGSSRLLAVGHPYYSVTKDNTKTNIPKVSAYQYRVFRVRLPDPNKFGLPDTNIYNPDQERLVWACVGLEVGRGQPLGAGLSGHPLFNRLDDTESSNLANNNVIEDSRDNISVDGKQTQLCIVGCTPAMGEHWTKGAVCKSTQVTTGDCPPLALINTPIEDGDMIDTGFGAMDFKVLQESKAEVPLDIVQSTCKYPDYLKMSADAYGDSMWFYLRREQLFARHYFNRAGKVGETIPAELYLKGSNGREPPPSSVYVATPSGSMITSEAQLFNKPYWLQRAQGHNNGICWGNQLFVTVVDTTRSTNMTISTATEQLSKYDARKINQYLRHVEEYELQFVFQLCKITLSAEVMAYLHNMNANLLEDWNIGLSPPVATSLEDKYRYVRSTAITCQREQPPTEKQDPLAKYKFWDVNLQDSFSTDLDQFPLGRKFLLQAGLKAKPKLKRAAPTSTRTSSAKRKKVKK

SEQ ID NO: 137 - DNA, 1498 bp, Artificial sequence
  5604 Nucleotide sequence of chimeric HPV type 56 L1 protein
atggctacctggagaccatctgagaacaaggtctacctgcctccaacacctgtgagcaaggtggtggctacagactcctatgtgaagaggaccagcatcttctaccatgctggctccagcagactgctggctgtgggacacccatactactctgtgaccaaggacaacaccaagaccaacatcccaaaggtgtctgcctaccaatacagggtgttcagggtgagactgcctgacccaaacaagtttggactgcctgacaccaacatctacaaccctgaccaggagagactggtgtgggcttgtgtgggattggaggtgggcaggggacaaccactgggagcaggactgtctggacacccactgttcaacagactggatgacacagagtccagcaacctggctaacaacaatgtgattgaggacagcagggacaacatctctgtggatggcaagcagacccaactttgtattgtgggctgtactcctgctatgggagaacactggaccaagggagcagtgtgtaagagcacccaggtgaccacaggagactgtcctccactggctctgataaacacaccaattgaggatggagatatgattgacacaggctttggagctatggacttcaaggtgctccaagagagcaaggctgaggtgccactggacattgtccagagcacttgtaaataccctgactacctgaaaatgagtgctgatgcctatggagacagtatgtggttctacctgaggagggaacaactttttgccagacactacttcaacagggctggcaaggtgggagagaccatccctgctgaactctacctgaaaggcagcaatggcagggaacctcctccatcctctgtctatgtggctacaccatctggcagtatgattacctctgaggctcaacttttcaacaagccatactggctccaaagggctcaaggacacaacaatggcatctgttggggcaaccaactttttgtgacagtggtggacaccaccaggagcaccaatatgaccatcagcacagccacagaacaacttagcaaatatgatgccaggaagataaaccaatacctgaggcatgtggaggaatatgaactccaatttgtgttccaactttgtaagattaccctgtctgctgaggtgatggcttacctgcacaatatgaatgccaacctgttggaggactggaacattggactgagccctcctgtggctacctccttggaggacaaatacagatatgtgaggagcacagccatcacttgtcagagggaacaacctccaacagagaagcaggacccactggctaaatacaagttctgggatgtgaacctccaagactccttcagcacagacctggaccagtttccactgggcaggaagttcctgctccaagcaggactgaaagccaagccaaaactgaaaagggctgccccaaccagcaccaggacctcctctgccaagaggaagaaggtgaagaagtaaa

SEQ ID NO: 138 - DNA, 1519 bp, Artificial sequence
  5605 Synthetic HPV56 L1 gene
ctgggtaccatggctacctggagaccatctgagaacaaggtctacctgcctccaacacctgtgagcaaggtggtggctacagactcctatgtgaagaggaccagcatcttctaccatgctggctccagcagactgctggctgtgggacacccatactactctgtgaccaaggacaacaccaagaccaacatcccaaaggtgtctgcctaccaatacagggtgttcagggtgagactgcctgacccaaacaagtttggactgcctgacaccaacatctacaaccctgaccaggagagactggtgtgggcttgtgtgggattggaggtgggcaggggacaaccactgggagcaggactgtctggacacccactgttcaacagactggatgacacagagtccagcaacctggctaacaacaatgtgattgaggacagcagggacaacatctctgtggatggcaagcagacccaactttgtattgtgggctgtactcctgctatgggagaacactggaccaagggagcagtgtgtaagagcacccaggtgaccacaggagactgtcctccactggctctgataaacacaccaattgaggatggagatatgattgacacaggctttggagctatggacttcaaggtgctccaagagagcaaggctgaggtgccactggacattgtccagagcacttgtaaataccctgactacctgaaaatgagtgctgatgcctatggagacagtatgtggttctacctgaggagggaacaactttttgccagacactacttcaacagggctggcaaggtgggagagaccatccctgctgaactctacctgaaaggcagcaatggcagggaacctcctccatcctctgtctatgtggctacaccatctggcagtatgattacctctgaggctcaacttttcaacaagccatactggctccaaagggctcaaggacacaacaatggcatctgttggggcaaccaactttttgtgacagtggtggacaccaccaggagcaccaatatgaccatcagcacagccacagaacaacttagcaaatatgatgccaggaagataaaccaatacctgaggcatgtggaggaatatgaactccaatttgtgttccaactttgtaagattaccctgtctgctgaggtgatggcttacctgcacaatatgaatgccaacctgttggaggactggaacattggactgagccctcctgtggctacctccttggaggacaaatacagatatgtgaggagcacagccatcacttgtcagagggaacaacctccaacagagaagcaggacccactggctaaatacaagttctgggatgtgaacctccaagactccttcagcacagacctggaccagtttccactgggcaggaagttcctgatgcaacttggcaccaggagcaagcctgctgtggctaccagcaagaagaggtctgccccaaccagcaccagcacacctgccaagaggaagaggaggtaaactcgagctc

SEQ ID NO: 139 - DNA, 1519 bp, Artificial sequence; identical to SEQ ID NO: 6
  5606 Synthetic HPV33 L1 gene

SEQ ID NO: 140 - DNA, 33 bp, Artificial sequence
  5607 HPV56L1 F1
cttggtaccatggctacctggagaccatctgag

SEQ ID NO: 141 - DNA, 31 bp, Artificial sequence
  5608 HPV56L1 R1
ctgcttggagcaggaacttcctgcccagtgg

SEQ ID NO: 142 - DNA, 1420 bp, Artificial sequence
  5609 HPV56L1 amplified sequence 1
cttggtaccatggctacctggagaccatctgagaacaaggtctacctgcctccaacacctgtgagcaaggtggtggctacagactcctatgtgaagaggaccagcatcttctaccatgctggctccagcagactgctggctgtgggacacccatactactctgtgaccaaggacaacaccaagaccaacatcccaaaggtgtctgcctaccaatacagggtgttcagggtgagactgcctgacccaaacaagtttggactgcctgacaccaacatctacaaccctgaccaggagagactggtgtgggcttgtgtgggattggaggtgggcaggggacaaccactgggagcaggactgtctggacacccactgttcaacagactggatgacacagagtccagcaacctggctaacaacaatgtgattgaggacagcagggacaacatctctgtggatggcaagcagacccaactttgtattgtgggctgtactcctgctatgggagaacactggaccaagggagcagtgtgtaagagcacccaggtgaccacaggagactgtcctccactggctctgataaacacaccaattgaggatggagatatgattgacacaggctttggagctatggacttcaaggtgctccaagagagcaaggctgaggtgccactggacattgtccagagcacttgtaaataccctgactacctgaaaatgagtgctgatgcctatggagacagtatgtggttctacctgaggagggaacaactttttgccagacactacttcaacagggctggcaaggtgggagagaccatccctgctgaactctacctgaaaggcagcaatggcagggaacctcctccatcctctgtctatgtggctacaccatctggcagtatgattacctctgaggctcaacttttcaacaagccatactggctccaaagggctcaaggacacaacaatggcatctgttggggcaaccaactttttgtgacagtggtggacaccaccaggagcaccaatatgaccatcagcacagccacagaacaacttagcaaatatgatgccaggaagataaaccaatacctgaggcatgtggaggaatatgaactccaatttgtgttccaactttgtaagattaccctgtctgctgaggtgatggcttacctgcacaatatgaatgccaacctgttggaggactggaacattggactgagccctcctgtggctacctccttggaggacaaatacagatatgtgaggagcacagccatcacttgtcagagggaacaacctccaacagagaagcaggacccactggctaaatacaagttctgggatgtgaacctccaagactccttcagcacagacctggaccagtttccactgggcaggaagttcctgctccaagcag

SEQ ID NO: 143 - DNA, 36 bp, Artificial sequence
  5610 HPV56L1 F2
gaagttcctgctccaagcaggactgaaagccaagcc

SEQ ID NO: 144 - DNA, 36 bp, Artificial sequence; identical to SEQ ID NO: 37
  5611 HPV56L1 R2

SEQ ID NO: 145 - DNA, 116 bp, Artificial sequence
  5612 HPV56L1 amplified sequence 2
gaagttcctgctccaagcaggactgaaagccaagccaaaactgaaaagggctgccccaaccagcaccaggacctcctctgccaagaggaagaaggtgaagaagtaaatctagacag

SEQ ID NO: 146 - protein, 38 aa, Homo sapiens; identical to SEQ ID NO: 13
  5613 Amino acid sequence of HPV type 59 L1 protein aa 471-508

SEQ ID NO: 147 - protein, 473 aa, Homo sapiens
  5801 Amino acid sequence of HPV type 58 L1 protein aa 1-473
MSVWRPSEATVYLPPVPVSKVVSTDEYVSRTSIYYYAGSSRLLAVGNPYFSIKSPNNNKKVLVPKVSGLQYRVFRVRLPDPNKFGFPDTSFYNPDTQRLVWACVGLEIGRGQPLGVGVSGHPYLNKFDDTETSNRYPAQPGSDNRECLSMDYKQTQLCLIGCKPPTGEHWGKGVACNNNAAATDCPPLELFNSIIEDGDMVDTGFGCMDFGTLQANKSDVPIDICNSTCKYPDYLKMASEPYGDSLFFFLRREQMFVRHFFNRAGKLGEAVPDDLYIKGSGNTAVIQSSAFFPTPSGSIVTSESQLFNKPYWLQRAQGHNNGICWGNQLFVTVVDTTRSTNMTLCTEVTKEGTYKNDNFKEYVRHVEEYDLQFVFQLCKITLTAEIMTYIHTMDSNILEDWQFGLTPPPSASLQDTYRFVTSQAITCQKTAPPKEKEDPLNKYTFWEVNLKEKFSADLDQFPLGRKFLLQSGL

SEQ ID NO: 148 - protein, 26 aa, Homo sapiens
  5802 Amino acid sequence of HPV type 33 L1 protein aa 474-499
KAKPKLKRAAPTSTRTSSAKRKKVKK

SEQ ID NO: 149 - protein, 499 aa, Artificial sequence
  5803 Amino acid sequence of chimeric HPV type 58 L1 protein
MSVWRPSEATVYLPPVPVSKVVSTDEYVSRTSIYYYAGSSRLLAVGNPYFSIKSPNNNKKVLVPKVSGLQYRVFRVRLPDPNKFGFPDTSFYNPDTQRLVWACVGLEIGRGQPLGVGVSGHPYLNKFDDTETSNRYPAQPGSDNRECLSMDYKQTQLCLIGCKPPTGEHWGKGVACNNNAAATDCPPLELFNSIIEDGDMVDTGFGCMDFGTLQANKSDVPIDICNSTCKYPDYLKMASEPYGDSLFFFLRREQMFVRHFFNRAGKLGEAVPDDLYIKGSGNTAVIQSSAFFPTPSGSIVTSESQLFNKPYWLQRAQGHNNGICWGNQLFVTVVDTTRSTNMTLCTEVTKEGTYKNDNFKEYVRHVEEYDLQFVFQLCKITLTAEIMTYIHTMDSNILEDWQFGLTPPPSASLQDTYRFVTSQAITCQKTAPPKEKEDPLNKYTFWEVNLKEKFSADLDQFPLGRKFLLQSGLKAKPKLKRAAPTSTRTSSAKRKKVKK

SEQ ID NO: 150 - DNA, 1501 bp, Artificial sequence
  5804 Nucleotide sequence of chimeric HPV type 58 L1 protein
atgagcgtgtggaggcccagcgaggccaccgtgtacctgccccccgtgcccgtgagcaaggtggtgagcaccgacgagtacgtgagcaggaccagcatctactactacgccggcagcagcaggctgctggccgtgggcaacccctacttcagcatcaagagccccaacaacaacaagaaggtgctggtgcccaaggtgagcggcctgcagtacagggtgttcagggtgaggctgcccgaccccaacaagttcggcttccccgacaccagcttctacaaccccgacacccagaggctggtgtgggcctgcgtgggcctggagatcggcaggggccagcccctgggcgtgggcgtgagcggccacccctacctgaacaagttcgacgacaccgagaccagcaacaggtaccccgcccagcccggcagcgacaacagggagtgcctgagcatggactacaagcagacccagctgtgcctgatcggctgcaagccccccaccggcgagcactggggcaagggcgtggcctgcaacaacaacgccgccgccaccgactgcccccccctggagctgttcaacagcatcatcgaggacggcgacatggtggacaccggcttcggctgcatggacttcggcaccctgcaggccaacaagagcgacgtgcccatcgacatctgcaacagcacctgcaagtaccccgactacctgaagatggccagcgagccctacggcgacagcctgttcttcttcctgaggagggagcagatgttcgtgaggcacttcttcaacagggccggcaagctgggcgaggccgtgcccgacgacctgtacatcaagggcagcggcaacaccgccgtgatccagagcagcgccttcttccccacccccagcggcagcatcgtgaccagcgagagccagctgttcaacaagccctactggctgcagagggcccagggccacaacaacggcatctgctggggcaaccagctgttcgtgaccgtggtggacaccaccaggagcaccaacatgaccctgtgcaccgaggtgaccaaggagggcacctacaagaacgacaacttcaaggagtacgtgaggcacgtggaggagtacgacctgcagttcgtgttccagctgtgcaagatcaccctgaccgccgagatcatgacctacatccacaccatggacagcaacatcctggaggactggcagttcggcctgacccccccccccagcgccagcctgcaggacacctacaggttcgtgaccagccaggccatcacctgccagaagaccgccccccccaaggagaaggaggaccccctgaacaagtacaccttctgggaggtgaacctgaaggagaagttcagcgccgacctggaccagttccccctgggcaggaagttcctgctgcagagcggcctgaaagccaagccaaaactgaaaagggctgccccaaccagcaccaggacctcctctgccaagaggaagaaggtgaagaagtaaa

SEQ ID NO: 151 - DNA, 1516 bp, Artificial sequence
  5805 Synthetic HPV58 L1 gene
ctgggtaccatgagcgtgtggaggcccagcgaggccaccgtgtacctgccccccgtgcccgtgagcaaggtggtgagcaccgacgagtacgtgagcaggaccagcatctactactacgccggcagcagcaggctgctggccgtgggcaacccctacttcagcatcaagagccccaacaacaacaagaaggtgctggtgcccaaggtgagcggcctgcagtacagggtgttcagggtgaggctgcccgaccccaacaagttcggcttccccgacaccagcttctacaaccccgacacccagaggctggtgtgggcctgcgtgggcctggagatcggcaggggccagcccctgggcgtgggcgtgagcggccacccctacctgaacaagttcgacgacaccgagaccagcaacaggtaccccgcccagcccggcagcgacaacagggagtgcctgagcatggactacaagcagacccagctgtgcctgatcggctgcaagccccccaccggcgagcactggggcaagggcgtggcctgcaacaacaacgccgccgccaccgactgcccccccctggagctgttcaacagcatcatcgaggacggcgacatggtggacaccggcttcggctgcatggacttcggcaccctgcaggccaacaagagcgacgtgcccatcgacatctgcaacagcacctgcaagtaccccgactacctgaagatggccagcgagccctacggcgacagcctgttcttcttcctgaggagggagcagatgttcgtgaggcacttcttcaacagggccggcaagctgggcgaggccgtgcccgacgacctgtacatcaagggcagcggcaacaccgccgtgatccagagcagcgccttcttccccacccccagcggcagcatcgtgaccagcgagagccagctgttcaacaagccctactggctgcagagggcccagggccacaacaacggcatctgctggggcaaccagctgttcgtgaccgtggtggacaccaccaggagcaccaacatgaccctgtgcaccgaggtgaccaaggagggcacctacaagaacgacaacttcaaggagtacgtgaggcacgtggaggagtacgacctgcagttcgtgttccagctgtgcaagatcaccctgaccgccgagatcatgacctacatccacaccatggacagcaacatcctggaggactggcagttcggcctgacccccccccccagcgccagcctgcaggacacctacaggttcgtgaccagccaggccatcacctgccagaagaccgccccccccaaggagaaggaggaccccctgaacaagtacaccttctgggaggtgaacctgaaggagaagttcagcgccgacctggaccagttccccctgggcaggaagttcctgctgcagagcggcctgaaggccaagcccaggctgaagaggagcgcccccaccaccagggcccccagcaccaagaggaagaaggtgaagaagtaaactcgagctc

SEQ ID NO: 152 - DNA, 1519 bp, Artificial sequence; identical to SEQ ID NO: 6
  5806 Synthetic HPV33 L1 gene

SEQ ID NO: 153 - DNA, 34 bp, Artificial sequence; identical to SEQ ID NO: 127
  5807 HPV58L1 F1

SEQ ID NO: 154 - DNA, 36 bp, Artificial sequence
  5808 HPV58L1 R1
gcttggctttcaggccgctctgcagcaggaacttcc

SEQ ID NO: 155 - DNA, 1438 bp, Artificial sequence
  5809 HPV58L1 amplified sequence 1
cttggtaccatgagcgtgtggaggcccagcgaggccaccgtgtacctgccccccgtgcccgtgagcaaggtggtgagcaccgacgagtacgtgagcaggaccagcatctactactacgccggcagcagcaggctgctggccgtgggcaacccctacttcagcatcaagagccccaacaacaacaagaaggtgctggtgcccaaggtgagcggcctgcagtacagggtgttcagggtgaggctgcccgaccccaacaagttcggcttccccgacaccagcttctacaaccccgacacccagaggctggtgtgggcctgcgtgggcctggagatcggcaggggccagcccctgggcgtgggcgtgagcggccacccctacctgaacaagttcgacgacaccgagaccagcaacaggtaccccgcccagcccggcagcgacaacagggagtgcctgagcatggactacaagcagacccagctgtgcctgatcggctgcaagccccccaccggcgagcactggggcaagggcgtggcctgcaacaacaacgccgccgccaccgactgcccccccctggagctgttcaacagcatcatcgaggacggcgacatggtggacaccggcttcggctgcatggacttcggcaccctgcaggccaacaagagcgacgtgcccatcgacatctgcaacagcacctgcaagtaccccgactacctgaagatggccagcgagccctacggcgacagcctgttcttcttcctgaggagggagcagatgttcgtgaggcacttcttcaacagggccggcaagctgggcgaggccgtgcccgacgacctgtacatcaagggcagcggcaacaccgccgtgatccagagcagcgccttcttccccacccccagcggcagcatcgtgaccagcgagagccagctgttcaacaagccctactggctgcagagggcccagggccacaacaacggcatctgctggggcaaccagctgttcgtgaccgtggtggacaccaccaggagcaccaacatgaccctgtgcaccgaggtgaccaaggagggcacctacaagaacgacaacttcaaggagtacgtgaggcacgtggaggagtacgacctgcagttcgtgttccagctgtgcaagatcaccctgaccgccgagatcatgacctacatccacaccatggacagcaacatcctggaggactggcagttcggcctgacccccccccccagcgccagcctgcaggacacctacaggttcgtgaccagccaggccatcacctgccagaagaccgccccccccaaggagaaggaggaccccctgaacaagtacaccttctgggaggtgaacctgaaggagaagttcagcgccgacctggaccagttccccctgggcaggaagttcctgctgcagagcggcctgaaagccaagc

SEQ ID NO: 156 - DNA, 35 bp, Artificial sequence
  5810 HPV58L1 F2
gagcggcctgaaagccaagccaaaactgaaaaggg

SEQ ID NO: 157 - DNA, 36 bp, Artificial sequence; identical to SEQ ID NO: 37
  5811 HPV58L1 R2

SEQ ID NO: 158 - DNA, 101 bp, Artificial sequence
  5812 HPV58L1 amplified sequence 2
gagcggcctgaaagccaagccaaaactgaaaagggctgccccaaccagcaccaggacctcctctgccaagaggaagaaggtgaagaagtaaatctagacag

SEQ ID NO: 159 - protein, 38 aa, Homo sapiens; identical to SEQ ID NO: 13
  5813 Amino acid sequence of HPV type 59 L1 protein aa 471-508

SEQ ID NO: 160 - protein, 508 aa, Homo sapiens
  5901 Amino acid sequence of HPV type 59 L1 protein
MALWRSSDNKVYLPPPSVAKVVSTDEYVTRTSIFYHAGSSRLLTVGHPYFKVPKGGNGRQDVPKVSAYQYRVFRVKLPDPNKFGLPDNTVYDPNSQRLVWACVGVEIGRGQPLGVGLSGHPLYNKLDDTENSHVASAVDTKDTRDNVSVDYKQTQLCIIGCVPAIGEHWTKGTACKPTTVVQGDCPPLELINTPIEDGDMVDTGYGAMDFKLLQDNKSEVPLDICQSICKYPDYLQMSADAYGDSMFFCLRREQVFARHFWNRSGTMGDQLPESLYIKGTDIRANPGSYLYSPSPSGSVVTSDSQLFNKPYWLHKAQGLNNGICWHNQLFLTVVDTTRSTNLSVCASTTSSIPNVYTPTSFKEYARHVEEFDLQFIFQLCKITLTTEVMSYIHNMNTTILEDWNFGVTPPPTASLVDTYRFVQSAAVTCQKDTAPPVKQDPYDKLKFWPVDLKERFSADLDQFPLGRKFLLQLGARPKPTIGPRKRAAPAPTSTPSPKRVKRRKSSRK

SEQ ID NO: 161 - DNA, 1528 bp, Homo sapiens
  5902 Nucleotide sequence of HPV type 59 L1 protein
atggctctgtggaggtcctctgacaacaaggtctacctgcctcctccatctgtggctaaggtggtgagcacagatgaatatgtgaccaggaccagcatcttctaccatgctggctccagcagactgctgacagtgggacacccatacttcaaggtgccaaagggaggcaatggcagacaggatgtgccaaaggtgtctgcctaccaatacagggtgttcagggtgaaactgcctgacccaaacaagtttggactgcctgacaacacagtctatgacccaaacagccagagactggtgtgggcttgtgtgggagtggagattggcaggggacaaccactgggagtgggactgtctggacacccactctacaacaaactggatgacacagagaactctcatgtggcatctgctgtggacaccaaggacaccagggacaatgtgtctgtggactacaagcagacccaactttgtatcattggctgtgtgcctgccattggagaacactggaccaagggcacagcctgtaagccaaccacagtggtccagggagactgtcctccattggaactgataaacacaccaattgaggatggagatatggtggacacaggctatggagctatggacttcaaactgctccaagacaacaagtctgaggtgccactggacatctgtcagagcatctgtaaataccctgactacctccaaatgagtgctgatgcctatggagacagtatgttcttctgtctgaggagggaacaggtgtttgccagacacttctggaacaggtctggcacaatgggagaccaacttcctgagtccctctacatcaagggcacagacatcagggctaaccctggctcctacctctacagcccaagcccatctggctctgtggtgacctctgacagccaacttttcaacaagccatactggctgcacaaggctcaaggactgaacaatggcatctgttggcacaaccaacttttcctgacagtggtggacaccaccaggagcaccaacctgtctgtgtgtgccagcaccacctccagcatcccaaatgtctacacaccaacctccttcaaggaatatgccaggcatgtggaggagtttgacctccaattcatcttccaactttgtaagattaccctgaccacagaggtgatgagttacatccacaatatgaacaccaccatcttggaggactggaactttggagtgacacctcctccaacagcctccctggtggacacctacaggtttgtccagtctgctgctgtgacttgtcagaaggacacagcccctcctgtgaagcaggacccatatgacaaactgaagttctggcctgtggacctgaaagagaggttctctgctgacctggaccagtttccactgggcaggaagttcctgctccaacttggagccagaccaaagccaaccattggaccaaggaagagggctgcccctgccccaaccagcacaccaagcccaaagagggtgaagaggaggaagtccagcaggaagtaaa

SEQ ID NO: 162 - DNA, 1546 bp, Artificial sequence; identical to SEQ ID NO: 87
  5903 Synthetic HPV59 L1 gene